European Patent Specification EP 3 830 120 B1, published May 24, 2023. Title: Novel fusion protein specific for CD137 and PD-L1. Applicant: Pieris Pharmaceuticals GmbH LES LABORATOIRES SERVIER. The sequence listing filed with the application follows.

SEQUENCE LISTING (148 sequences)

SEQ ID NO: 1 - protein, 158 aa, Homo sapiens
HHLLASDEEIQDVSGTWYLKAMTVDREFPEMNLESVTPMTLTTLEGGNLEAKVTMLISGRCQEVKAVLEKTDEPGKYTADGGKHVAYIIRSHVKDHYIFYCEGELHGKPVRGVKLVGRDPKNNLEALEDFEKAAGARGLSTESILIPRQSETCSPGSD

SEQ ID NO: 2 - protein, 178 aa, Homo sapiens
QDSTSDLIPAPPLSKVPLQQNFQDNQFQGKWYVVGLAGNAILREDKDPQKMYATIYELKEDKSYNVTSVLFRKKKCDYWIRTFVPGCQPGEFTLGNIKSYPGLTSYLVRVVSTNYNQHAMVFFKKVSQNREYFKITLYGRTKELTSELKENFIRFSKSLGLPENHIVFPVPIDQCIDG

SEQ ID NO: 3 - protein, 178 aa, Artificial Sequence
  lipocalin mutein
QDSTSDLIPAPPLSKVPLQQNFQDNQFHGKWYVVGLAGNAILREDKDPQKMYATIYELKEDKSYNVTSVLFRKKKCDYWIRTFVPGSQPGEFTLGNIKSYPGLTSYLVRVVSTNYNQHAMVFFKKVSQNREYFKITLYGRTKELTSELKENFIRFSKSLGLPENHIVFPVPIDQCIDG

SEQ ID NO: 4 - protein, 152 aa, Artificial Sequence
  lipocalin mutein
ASDEEIQDVSGTWYLKAMTVDRECPEMNLESVTPMTLTTLEGGNLEAKVTMLISGRSQEVKAVLEKTDEPGKYTADGGKHVAYIIRSHVKDHYIFYSEGECHGKPVPGVWLVGRDPKNNLEALEDFEKAAGARGLSTESILIPRQSETSSPG

SEQ ID NO: 5 - protein, 4 aa, Homo sapiens
HHLL

SEQ ID NO: 6 - protein, 272 aa, Homo sapiens
FTVTVPKDLYVVEYGSNMTIECKFPVEKQLDLAALIVYWEMEDKNIIQFVHGEEDLKVQHSSYRQRARLLKDQLSLGNAALQITDVKLQDAGVYRCMISYGGADYKRITVKVNAPYNKINQRILVVDPVTSEHELTCQAEGYPKAEVIWTSSDHQVLSGKTTTTNSKREEKLFNVTSTLRINTTTNEIFYCTFRRLDPEENHTAELVIPELPLAHPPNERTHLVILGAILLCLGVALTFIFRLRKGRMMDVKKCGIQDTNSKKQSDTHLEET

SEQ ID NO: 7 - protein, 232 aa, Homo sapiens
LQDPCSNCPAGTFCDNNRNQICSPCPPNSFSSAGGQRTCDICRQCKGVFRTRKECSSTSNAECDCTPGFHCLGAGCSMCEQDCKQGQELTKKGCKDCCFGTFNDQKRGICRPWTNCSLDGKSVLVNGTKERDVVCGPSPADLSPGASSVTPPAPAREPGHSPQIISFFLALTSTALLFLLFFLTLRFSVVKRGRKKLLYIFKQPFMRPVQTTQEEDGCSCRFPEEEEGGCEL

SEQ ID NO: 8 - protein, 272 aa, Macaca fascicularis
FTVTVPKDLYVVEYGSNMTIECKFPVEKQLDLTSLIVYWEMEDKNIIQFVHGEEDLKVQHSNYRQRAQLLKDQLSLGNAALRITDVKLQDAGVYRCMISYGGADYKRITVKVNAPYNKINQRILVVDPVTSEHELTCQAEGYPKAEVIWTSSDHQVLSGKTTTTNSKREEKLLNVTSTLRINTTANEIFYCIFRRLDPEENHTAELVIPELPLALPPNERTHLVILGAIFLLLGVALTFIFYLRKGRMMDMKKSGIRVTNSKKQRDTQLEET

SEQ ID NO: 9 - protein, 231 aa, Macaca fascicularis
LQDLCSNCPAGTFCDNNRSQICSPCPPNSFSSAGGQRTCDICRQCKGVFKTRKECSSTSNAECDCISGYHCLGAECSMCEQDCKQGQELTKKGCKDCCFGTFNDQKRGICRPWTNCSLDGKSVLVNGTKERDVVCGPSPADLSPGASSATPPAPAREPGHSPQIIFFLALTSTVVLFLLFFLVLRFSVVKRSRKKLLYIFKQPFMRPVQTTQEEDGCSCRFPEEEEGGCEL

SEQ ID NO: 10 - protein, 4 aa, Artificial Sequence
  cleavage site
IEGR

SEQ ID NO: 11 - protein, 10 aa, Artificial Sequence
  fusion peptide
SAWSHPQFEK

SEQ ID NO: 12 - protein, 8 aa, Artificial Sequence
  Step-Tag II peptide
WSHPQFEK

SEQ ID NO: 13 - protein, 15 aa, Artificial Sequence
  linker
GGGGSGGGGSGGGGS

SEQ ID NO: 14 - protein, 18 aa, Artificial Sequence
  linker
PSTPPTNSSSTPPTPSPS

SEQ ID NO: 15 - protein, 14 aa, Artificial Sequence
  linker
GGSGNSSGSGGSPV

SEQ ID NO: 16 - protein, 20 aa, Artificial Sequence
  linker
ASPAAPAPASPAAPAPSAPA

SEQ ID NO: 17 - protein, 66 aa, Artificial Sequence
  linker
AGSGGSGGSGGSPVPSTPPTPSPSTPPTPSPSGGSGNSSGSGGSPVPSTPPTPSPSTPPTPSPSAS

SEQ ID NO: 18 - protein, 32 aa, Artificial Sequence
  linker
PSTPPTPSPSTPPTPSPSGGSGNSSGSGGSPV

SEQ ID NO: 19 - protein, 74 aa, Artificial Sequence
  linker
AGSGGSGGSGGSPVPSTPPTNSSSTPPTPSPSPVPSTPPTNSSSTPPTPSPSPVPSTPPTNSSSTPPTPSPSAS

SEQ ID NO: 20 - protein, 40 aa, Artificial Sequence
  linker
ASPAAPAPASPAAPAPSAPAASPAAPAPASPAAPAPSAPA

SEQ ID NO: 21 - protein, 10 aa, Artificial Sequence
  linker
VDDIEGRMDE

SEQ ID NO: 22 - protein, 11 aa, Artificial Sequence
  linker
ENLYFQGRMDE

SEQ ID NO: 23 - protein, 10 aa, Artificial Sequence
  linker
GGGGSGGGGS

SEQ ID NO: 24 - protein, 327 aa, Homo sapiens
ASTKGPSVFPLAPCSRSTSESTAALGCLVKDYFPEPVTVSWNSGALTSGVHTFPAVLQSSGLYSLSSVVTVPSSSLGTKTYTCNVDHKPSNTKVDKRVESKYGPPCPSCPAPEFLGGPSVFLFPPKPKDTLMISRTPEVTCVVVDVSQEDPEVQFNWYVDGVEVHNAKTKPREEQFNSTYRVVSVLTVLHQDWLNGKEYKCKVSNKGLPSSIEKTISKAKGQPREPQVYTLPPSQEEMTKNQVSLTCLVKGFYPSDIAVEWESNGQPENNYKTTPPVLDSDGSFFLYSRLTVDKSRWQEGNVFSCSVMHEALHNHYTQKSLSLSLGK

SEQ ID NO: 25 - protein, 214 aa, Homo sapiens
EIVLTQSPATLSLSPGERATLSCRASQSVSSYLAWYQQKPGQAPRLLIYDASNRATGIPARFSGSGSGTDFTLTISSLEPEDFAVYYCQQSSNWPRTFGQGTKVEIKRTVAAPSVFIFPPSDEQLKSGTASVVCLLNNFYPREAKVQWKVDNALQSGNSQESVTEQDSKDSTYSLSSTLTLSKADYEKHKVYACEVTHQGLSSPVTKSFNRGEC

SEQ ID NO: 26 - protein, 448 aa, Artificial Sequence
  antibody heavy chain
EVQLVESGGGLVQPGGSLRLSCAASGFTFSDSWIHWVRQAPGKGLEWVAWISPYGGSTYYADSVKGRFTISADTSKNTAYLQMNSLRAEDTAVYYCARRHWPGGFDYWGQGTLVTVSSASTKGPSVFPLAPSSKSTSGGTAALGCLVKDYFPEPVTVSWNSGALTSGVHTFPAVLQSSGLYSLSSVVTVPSSSLGTQTYICNVNHKPSNTKVDKKVEPKSCDKTHTCPPCPAPELLGGPSVFLFPPKPKDTLMISRTPEVTCVVVDVSHEDPEVKFNWYVDGVEVHNAKTKPREEQYASTYRVVSVLTVLHQDWLNGKEYKCKVSNKALPAPIEKTISKAKGQPREPQVYTLPPSREEMTKNQVSLTCLVKGFYPSDIAVEWESNGQPENNYKTTPPVLDSDGSFFLYSKLTVDKSRWQQGNVFSCSVMHEALHNHYTQKSLSLSPGK

SEQ ID NO: 27 - protein, 214 aa, Artificial Sequence
  antibody light chain
DIQMTQSPSSLSASVGDRVTITCRASQDVSTAVAWYQQKPGKAPKLLIYSASFLYSGVPSRFSGSGSGTDFTLTISSLQPEDFATYYCQQYLYHPATFGQGTKVEIKRTVAAPSVFIFPPSDEQLKSGTASVVCLLNNFYPREAKVQWKVDNALQSGNSQESVTEQDSKDSTYSLSSTLTLSKADYEKHKVYACEVTHQGLSSPVTKSFNRGEC

SEQ ID NO: 28 - protein, 448 aa, Artificial Sequence
  antibody heavy chain
QVQLQQWGAGLLKPSETLSLTCAVYGGSFSGYYWSWIRQSPEKGLEWIGEINHGGYVTYNPSLESRVTISVDTSKNQFSLKLSSVTAADTAVYYCARDYGPGNYDWYFDLWGRGTLVTVSSASTKGPSVFPLAPCSRSTSESTAALGCLVKDYFPEPVTVSWNSGALTSGVHTFPAVLQSSGLYSLSSVVTVPSSSLGTKTYTCNVDHKPSNTKVDKRVESKYGPPCPPCPAPEFLGGPSVFLFPPKPKDTLMISRTPEVTCVVVDVSQEDPEVQFNWYVDGVEVHNAKTKPREEQFNSTYRVVSVLTVLHQDWLNGKEYKCKVSNKGLPSSIEKTISKAKGQPREPQVYTLPPSQEEMTKNQVSLTCLVKGFYPSDIAVEWESNGQPENNYKTTPPVLDSDGSFFLYSRLTVDKSRWQEGNVFSCSVMHEALHNHYTQKSLSLSLGK

SEQ ID NO: 29 - protein, 216 aa, Artificial Sequence
  antibody light chain
EIVLTQSPATLSLSPGERATLSCRASQSVSSYLAWYQQKPGQAPRLLIYDASNRATGIPARFSGSGSGTDFTLTISSLEPEDFAVYYCQQRSNWPPALTFGGGTKVEIKRTVAAPSVFIFPPSDEQLKSGTASVVCLLNNFYPREAKVQWKVDNALQSGNSQESVTEQDSKDSTYSLSSTLTLSKADYEKHKVYACEVTHQGLSSPVTKSFNRGEC

SEQ ID NO: 30 - protein, 228 aa, Artificial Sequence
  antibody fragment
ESKYGPPCPPCPAPEAAGGPSVFLFPPKPKDTLMISRTPEVTCVVVDVSQEDPEVQFNWYVDGVEVHNAKTKPREEQFNSTYRVVSVLTVLHQDWLNGKEYKCKVSNKGLPSSIEKTISKAKGQPREPQVYTLPPSQEEMTKNQVSLTCLVKGFYPSDIAVEWESNGQPENNYKTTPPVLDSDGSFFLYSRLTVDKSRWQEGNVFSCSVMHEALHNHYTQKSLSLSLG

SEQ ID NO: 31 - protein, 228 aa, Artificial Sequence
  antibody fragment
ESKYGPPCPPCPAPEFLGGPSVFLFPPKPKDTLMISRTPEVTCVVVDVSQEDPEVQFNWYVDGVEVHNAKTKPREEQFNSTYRVVSVLTVLHQDWLNGKEYKCKVSNKGLPSSIEKTISKAKGQPREPQVYTLPPSQEEMTKNQVSLTCLVKGFYPSDIAVEWESNGQPENNYKTTPPVLDSDGSFFLYSRLTVDKSRWQEGNVFSCSVMHEALHNHYTQKSLSLSLG

SEQ ID NO: 32 - protein, 228 aa, Artificial Sequence
  antibody fragment
ESKYGPPCPPCPAPEFLGGPSVFLFPPKPKDTLMISRTPEVTCVVVDVSQEDPEVQFNWYVDGVEVHNAKTKPREEQFNSTYRVVSVLTVLHQDWLNGKEYKCKVSNKGLPSSIEKTISKAKGQPREPQVYTLPPSQEEMTKNQVSLTCLVKGFYPSDIAVEWESNGQPENNYKTTPPVLDSDGSFFLYSRLTVDKSRWQEGNVFSCSVLHEALHSHYTQKSLSLSLG

SEQ ID NO: 33 - protein, 228 aa, Artificial Sequence
  antibody fragment
ESKYGPPCPPCPAPEFLGGPSVFLFPPKPKDTLYITREPEVTCVVVDVSQEDPEVQFNWYVDGVEVHNAKTKPREEQFNSTYRVVSVLTVLHQDWLNGKEYKCKVSNKGLPSSIEKTISKAKGQPREPQVYTLPPSQEEMTKNQVSLTCLVKGFYPSDIAVEWESNGQPENNYKTTPPVLDSDGSFFLYSRLTVDKSRWQEGNVFSCSVMHEALHNHYTQKSLSLSLG

SEQ ID NO: 34 - protein, 152 aa, Artificial Sequence
  lipocalin mutein
ASDEEIQDVSGTWYLKAMTVDEGCRPWNIFSVTPMTLTTLEGGNLEAKVTMAIDGPAQEVKAVLEKTDEPGKYTADGGKHVAYIIRSHVKDHYIFYSEGVCDGSPVPGVWLVGRDPKNNLEALEDFEKAAGARGLSTESILIPRQSETSSPG

SEQ ID NO: 35 - protein, 152 aa, Artificial Sequence
  lipocalin mutein
TSDEEIQDVSGTWYLKAMTVDEGCRPWNIFSVTPMTLTTLEGGNLEAKVTMAIDGPAQEVRAVLEKTDEPGKYTADGGKHDAYIIRSHVKDHYIFYSEGVCDGSPVPGVWLVGRDPENNLEALEDFEKTAGARGLSTESILIPRQSETSSPG

SEQ ID NO: 36 - protein, 152 aa, Artificial Sequence
  lipocalin mutein
ASDEEIQDVSGTWYLKAMTVDEGCRPWNIFSVTPMTLTTLEGGNLEAKVTMAIDGPAQEVNAVLEKTDEPGKYTADGGKHVAYIIRSHVRDHYIFYSEGVCDGSPVPGVWLVGRDPENNLEALEDFEKTAGARGLSTESILIPRQSETSSPG

SEQ ID NO: 37 - protein, 152 aa, Artificial Sequence
  lipocalin mutein
VSDEEIQDVSGTWYLKAMTVDEGCRPWNIFSVTPMTLTTLEGGNLEAKVTMAIDGPAQEVRAVLEKTDEPGKYTADGGKHVAYIIRSHVEDHYIFYSEGVCDGSPVPGVWLVGRDPENNLEALEDFEKTAGARGLSTESILIPRQSETSSPG

SEQ ID NO: 38 - protein, 152 aa, Artificial Sequence
  lipocalin mutein
ASDEEIQDVSGTWYLKAMTVDEGCRPWNIFSVTPMTLSTLEGGNLEAKVTMAIDGPAQEVKAVLEKTDEPGKYTADGGKHVAYIIRSHVKDHYIFYSEGVCDGSPVPGVWLVGRDPKNNLEALEDFEKAAGARGLSTESILIPRQIETSSPG

SEQ ID NO: 39 - protein, 152 aa, Artificial Sequence
  lipocalin mutein
ASDEEIQDVSGTWYLKAMTVDEGCRPWNIFSVTPMTLTTLEGGNLEAEVTMAIDGPAQEVKAVLEKADEPGKYTADGGKHVAYIIRSHVKDHYIFYSEGVCDGSPVPGVWLVGRDPKNNLEALEDFEKTAGARGLSTESILIPSQIETSSPG

SEQ ID NO: 40 - protein, 152 aa, Artificial Sequence
  lipocalin mutein
TSDEEIQDVSGTWYLKAMTVDEGCRPWNIFSVTPMTLTTLEDGNLEAKVTMAIDGPAQEVKAVLEKADEPGKYTADGGKHVAYIIRSHVKDHYIFYSEGVCDGSPVPGVWLVGRDPKNNLEALEDFEKAAGARGLSTESILIPRQIETSSPG

SEQ ID NO: 41 - protein, 178 aa, Artificial Sequence
  lipocalin mutein
QDSTSDLIPAPPLSKVPLQQNFQDNQFHGKWYVVGQAGNIKLREDKDPNKMMATIYELKEDKSYNVTGVTFDDKKCTYAISTFVPGSQPGEFTLGKIKSFPGHTSSLVRVVSTNYNQHAMVFFKFVFQNREEFYITLYGRTKELTSELKENFIRFSKSLGLPENHIVFPVPIDQCIDG

SEQ ID NO: 42 - protein, 178 aa, Artificial Sequence
  lipocalin mutein
QDSTSDLIPAPPLSKVPLQQNFQDNQFHGKWYVVGQAGNIRLREDKDPIKMMATIYELKEDKSYDVTMVKFDDKKCMYDIWTFVPGSQPGEFTLGKIKSFPGHTSSLVRVVSTNYNQHAMVFFKFVFQNREEFYITLYGRTKELTSELKENFIRFSKSLGLPENHIVFPVPIDQCIDG

SEQ ID NO: 43 - protein, 178 aa, Artificial Sequence
  lipocalin mutein
QDSTSDLIPAPPLSKVPLQQNFQDNQFHGKWYVVGQAGNIRLREDKDPNKMMATIYELKEDKSYDVTAVAFDDKKCTYDIWTFVPGSQPGEFTLGKIKSFPGHTSSLVRVVSTNYNQHAMVFFKFVFQNREEFYITLYGRTKELTSELKENFIRFSKSLGLPENHIVFPVPIDQCIDG

SEQ ID NO: 44 - protein, 178 aa, Artificial Sequence
  lipocalin mutein
QDSTSDLIPAPPLSKVPLQQNFQDNQFHGKWYVVGQAGNIKLREDKDPNKMMATIYELKEDKSYDVTAVAFDDKKCTYDIWTFVPGSQPGEFTLGKIKSFPGHTSSLVRVVSTNYNQHAMVFFKFVFQNREEFYITLYGRTKELTSELKENFIRFSKSLGLPENHIVFPVPIDQCIDG

SEQ ID NO: 45 - protein, 175 aa, Artificial Sequence
  lipocalin mutein
QDSTSDLIPAPPLSKVPLQQNFQDNQFHGKWYVVGQAGNIKLREDSKMMATIYELKEDKSYDVTGVSFDDKKCTYAIMTFVPGSQPGEFTLGKIKSFPGHTSSLVRVVSTNYNQHAMVFFKFVFQNREEFYITLYGRTKELTSELKENFIRFSKSLGLPENHIVFPVPIDQCIDG

SEQ ID NO: 46 - protein, 178 aa, Artificial Sequence
  lipocalin mutein
QDSTSDLIPAPPLSKVPLQQNFQDNQFHGKWYVVGQAGNIKLREDKDPVKMMATIYELKEDKSYDVTGVTFDDKKCRYDISTFVPGSQPGEFTFGKIKSFPGHTSSLVRVVSTNYNQHAMVFFKFVFQNREEFYITLYGRTKELTSELKENFIRFSKSLGLPENHIVFPVPIDQCIDG

SEQ ID NO: 47 - protein, 178 aa, Artificial Sequence
  lipocalin mutein
QDSTSDLIPAPPLSKVPLQQNFQDNQFHGKWYVVGQAGNIRLREDKDPHKMMATIYELKEDKSYDVTGVTFDDKKCTYAISTFVPGSQPGEFTLGKIKSFPGHTSSLVRVVSTNYNQHAMVFFKFVFQNREEFYITLYGRTKELTSELKENFIRFSKSLGLPENHIVFPVPIDQCIDG

SEQ ID NO: 48 - protein, 178 aa, Artificial Sequence
  lipocalin mutein
QDSTSDLIPAPPLSKVPLQQNFQDNQFHGKWYVVGQAGNIKLREDKDPNKMMATIYELKEDKSYDVTGVTFDDKKCTYAISTLVPGSQPGEFTFGKIKSFPGHTSSLVRVVSTNYNQHAMVFFKFVFQNREEFYITLYGRTKELTSELKENFIRFSKSLGLPENHIVFPVPIDQCIDG

SEQ ID NO: 49 - protein, 178 aa, Artificial Sequence
  lipocalin mutein
QDSTSDLIPAPPLSKVPLQQNFQDNQFHGKWYVVGQAGNIRLREDKDPSKMMATIYELKEDKSYDVTAVTFDDKKCNYAISTFVPGSQPGEFTLGKIKSFPGHTSSLVRVVSTNYNQHAMVFFKFVFQNREEFYITLYGRTKELTSELKENFIRFSKSLGLPENHIVFPVPIDQCIDG

SEQ ID NO: 50 - protein, 178 aa, Artificial Sequence
  lipocalin mutein
QDSTSDLIPAPPLSKVPLQQNFQDNQFHGKWYVVGMAGNNLLREDKDPHKMSATIYELKEDKSYNVTDVMFLDKKCQYIIWTFVPGSQPGEFTLGFIKSDPGHTSYLVRVVSTNYNQHAMVFFKSVIQNREWFGITLYGRTKELTSELKENFIRFSKSLGLPENHIVFPVPIDQCIDG

SEQ ID NO: 51 - protein, 178 aa, Artificial Sequence
  lipocalin mutein
QDSTSDLIPAPPLSKVPLQQNFQDNQFQGKWYVVGMAGNNLLREDKDPHKMSATIYELKEDKSYNVTDVMFLDKKCQYIIWTFVPGSQPGELTLGFIRSDLGHTSYLVRVVSTNYNQHAMVFFKSVIQNREWFGITLYGRTKELTSELKENFIRFSKSLGLPENHIVFPVPIDQCIDG

SEQ ID NO: 52 - protein, 178 aa, Artificial Sequence
  lipocalin mutein
QDSTSDLIPAPPLSKVPLQQNFQDYQFQGKWYVVGMAGNNLLREDKDPHKMGATIYELKEDKSYNVTDVMLLDKKCQYIIQTFVPGSQPGESTLGFIKSDPGHTSYLVRVVSTNYNQHAMVFFKSVIQNREWFGITLYGRTKELTSELKENFIRFSKSLGLPENHIVFPVPIDQCIDG

SEQ ID NO: 53 - protein, 178 aa, Artificial Sequence
  lipocalin mutein
QDSTSDLIPAPPLSKVPLQQNFQDNQFQGKWYVVGMAGNNLLREDKDPHKMGATIYELKEDKSYNVTDVMFLDKKCQHIIWTFVPGSQPGELTLGFIKSDPGHTSYLVRVVSTNYNQHAMVFFKSVIQNREWFGITLYGRTKELTSELKENFIRFSKSLGLPENHIVFPVPIDQCIDG

SEQ ID NO: 54 - protein, 178 aa, Artificial Sequence
  lipocalin mutein
QDSTSDLIPAPPLSKVPLQQNFQDDQFQGKWYVVGMAGNNLLREDKDPHKMGATIYELKEDKSYNVTDVMFLDKKCQYIIWTFVPGSQPGELTLGFIKSDPGHTSYLVRVVSTNYNQHAMVFFKSVIQNREWFGITLYGRTKELTSELKENFIRFSKSLGLPENHIVFPVPIDQCIDG

SEQ ID NO: 55 - protein, 178 aa, Artificial Sequence
  lipocalin mutein
QDSTSDLIPAPPLSKVPLQQNFQDNQFQGKWYIVGMAGNNLLREDKDPHKMGATIYELKEDKSYNVTDVMFLDKKCQYIIWTFVPGSQPGELTLGFIKSDPGHTSYLVRVVSTNYNQHAMVFFKSVIQNREWFGITLYGRTKELTSELKENFIRFSKSLGLPENHIVFPVPIDQCIDG

SEQ ID NO: 56 - protein, 178 aa, Artificial Sequence
  lipocalin mutein
QDSTSDLIPAPPLSKVPLQRNFQDNQFQGKWYVVGMAGNNLLRVDKDPHKMGATIYELKEDKSYNVTDVMFLDKKCQYIIWTFVPGSQPGELTLGFIKSDPGHTSYLVRVVSTNYNQHAMVYFKSVIQNREWFGITLYGRTKELTSELKENFIRFSKSLGLPENHIVFPVPIDQCIDG

SEQ ID NO: 57 - protein, 178 aa, Artificial Sequence
  lipocalin mutein
QDSTSDLIPAPPLSKVPLQQNFQDNQFQGKWYVVGMAGNNLLREDKDPHKMSATIYELKEDKSYNVTDVMFLDKKCQYINWPFVPGSQPGEFTLGFIKSDLGPTSYLVRVVSTNYNQHAMVFFKSVIQNREWFGITLYGRTKELTSELKENFIRFSKSLGLPENHIVFPVPIDQCIDG

SEQ ID NO: 58 - protein, 178 aa, Artificial Sequence
  lipocalin mutein
QDSTSDLIPAPPLSKVPLQQNFQDNQFQGKWYVVGMAGNNLLREDKDPHKMGATIYELNEDKSYNVTDVMFLDKKCQYIIWTFVPGSQPGELTLGFIKSDPGHTSYLVRVVSTNYNQHAMVFFKSVIQNREWFGITLYGRTKELTSELKENFIRFSKSLGLPENHIVFPVPIDQCIDG

SEQ ID NO: 59 - protein, 178 aa, Artificial Sequence
  lipocalin mutein
QDSTSDLIPAPPLSKVPLQQNFQDNQFQGKWYVVGMAGNNLLRDDKDPHKMSATIYELKEDKSYNVTDVMLLDKKCHYIIWTFVPGSQPGELTLGFIKSDPGHTSYLVRVVSTNYNQHAMVFFKSVIQNREWFGITLYGRTKELTSELKENFIRFSKSLGLPENHIVFPVPIDQCIDG

SEQ ID NO: 60 - protein, 8 aa, Artificial Sequence
  antibody heavy chain CDR1
GFSLSNYD

SEQ ID NO: 61 - protein, 7 aa, Artificial Sequence
  antibody heavy chain CDR2
IWTGGAT

SEQ ID NO: 62 - protein, 14 aa, Artificial Sequence
  antibody heavy chain CDR3
VRDSNYRYDEPFTY

SEQ ID NO: 63 - protein, 6 aa, Artificial Sequence
  antibody light chain CDR1
QSIGTN

SEQ ID NO: 64 - protein, 9 aa, Artificial Sequence
  antibody light chain CDR3
QQSNSWPYT

SEQ ID NO: 65 - protein, 8 aa, Artificial Sequence
  antibody heavy chain CDR1
GFDIKDTY

SEQ ID NO: 66 - protein, 8 aa, Artificial Sequence
  antibody heavy chain CDR2
IDPADGNT

SEQ ID NO: 67 - protein, 10 aa, Artificial Sequence
  antibody heavy chain CDR3
ARGLGAWFAS

SEQ ID NO: 68 - protein, 6 aa, Artificial Sequence
  antibody light chain CDR1
QDITNS

SEQ ID NO: 69 - protein, 9 aa, Artificial Sequence
  antibody light chain CDR3
QQGHTLPPT

SEQ ID NO: 70 - protein, 8 aa, Artificial Sequence
  antibody heavy chain CDR1
GFNIKDTY

SEQ ID NO: 71 - protein, 8 aa, Artificial Sequence
  antibody heavy chain CDR2
IDPANGNT

SEQ ID NO: 72 - protein, 17 aa, Artificial Sequence
  antibody heavy chain CDR3
SRGPPGGIGEYIYAMDY

SEQ ID NO: 73 - protein, 7 aa, Artificial Sequence
  antibody light chain CDR1
SSVSSSY

SEQ ID NO: 74 - protein, 9 aa, Artificial Sequence
  antibody light chain CDR3
HQYHRSPPT

SEQ ID NO: 75 - protein, 120 aa, Artificial Sequence
  antibody heavy chain variable region
QVQLKESGPGLVAPSQNLSITCTVSGFSLSNYDISWIRQPPGKGLEWLGVIWTGGATNYNSAFMSRLSISRDNSKSQVFLKMNSLQTDDTAIYYCVRDSNYRYDEPFTYWGQGTLVTVSA

SEQ ID NO: 76 - protein, 120 aa, Artificial Sequence
  antibody heavy chain variable region
QVQLQESGPGLVKPSENLSITCTVSGFSLSNYDISWIRQPPGKGLEWLGVIWTGGATNYNPAFKSRLTISRDNSKSQVSLKMSSLQAADTAVYYCVRDSNYRYDEPFTYWGQGTLVTVSS

SEQ ID NO: 77 - protein, 120 aa, Artificial Sequence
  antibody heavy chain variable region
QVQLQESGPGLVKPSETLSITCTVSGFSLSNYDISWIRQPPGKGLEWLGVIWTGGATNYNPALKSRLTISRDNSKNQVSLKMSSVTAADTAVYYCVRDSNYRYDEPFTYWGQGTLVTVSS

SEQ ID NO: 78 - protein, 117 aa, Artificial Sequence
  antibody heavy chain variable region
EVQLQQSGAELVKPGASVKLSCTASGFDIKDTYIHWVKQRPEQGLEWIGRIDPADGNTRYDPKFQDKTTITTDTSSNTAHLQLSSLTSEDTAVYYCARGLGAWFASWGQGTLVTVSA

SEQ ID NO: 79 - protein, 124 aa, Artificial Sequence
  antibody heavy chain variable region
EVQLQQSGAELVKPGASVKLSCTASGFNIKDTYMYWVKQRPEQGLEWIGRIDPANGNTKYDPKFQGKATITADTSANTAYLQLSSLTSEDTAVYYCSRGPPGGIGEYIYAMDYWGQGTSVTVSS

SEQ ID NO: 80 - protein, 106 aa, Artificial Sequence
  antibody light chain variable region
DILLTQSPAILSVSPGERVSLSCRASQSIGTNIHWFQQRTNGSPRLLIKYASESISGIPSRFSGSGSGTDFTLSINSVESEDIADYYCQQSNSWPYTFGGGTKLEI

SEQ ID NO: 81 - protein, 107 aa, Artificial Sequence
  antibody light chain variable region
EIVLTQSPDTLSVTPKEKVTLTCRASQSIGTNIHWFQQRPGQSPKLLIKYASESISGIPSRFSGSGSGTDFTLTINSVEAEDAATYYCQQSNSWPYTFGQGTKLEIK

SEQ ID NO: 82 - protein, 107 aa, Artificial Sequence
  antibody light chain variable region
EIVLTQSPDTLSVTPKEKVTLTCRASQSIGTNIHWFQQKPGQSPKLLIKYASESISGVPSRFSGSGSGTDFTLTINSVEAEDAATYYCQQSNSWPYTFGQGTKLEIK

SEQ ID NO: 83 - protein, 106 aa, Artificial Sequence
  antibody light chain variable region
DIQMTQTTSSLSASLGDRVTISCRASQDITNSLNWYQQKPDGTVKLLIHYTSRLHSGVPSRFSGSGSGTDYSLTISNLEQEDIATYFCQQGHTLPPTFGGGTKLEI

SEQ ID NO: 84 - protein, 107 aa, Artificial Sequence
  antibody light chain variable region
QIVLTQSPAIMSASLGERVTMTCTASSSVSSSYLHWYQQKPGSSPKLWIYSTSNLASGVPARFSGSGSGTSYSLTISSMEAEDAATYYCHQYHRSPPTFGGGTKLEI

SEQ ID NO: 85 - protein, 450 aa, Artificial Sequence
  antibody heavy chain
QVQLQESGPGLVKPSETLSITCTVSGFSLSNYDISWIRQPPGKGLEWLGVIWTGGATNYNPALKSRLTISRDNSKNQVSLKMSSVTAADTAVYYCVRDSNYRYDEPFTYWGQGTLVTVSSASTKGPSVFPLAPSSKSTSGGTAALGCLVKDYFPEPVTVSWNSGALTSGVHTFPAVLQSSGLYSLSSVVTVPSSSLGTQTYICNVNHKPSNTKVDKKVEPKSCDKTHTCPPCPAPEAAGAPSVFLFPPKPKDTLMISRTPEVTCVVVDVSHEDPEVKFNWYVDGVEVHNAKTKPREEQYNSTYRVVSVLTVLHQDWLNGKEYKCKVSNKALPAPIEKTISKAKGQPREPQVYTLPPSRDELTKNQVSLTCLVKGFYPSDIAVEWESNGQPENNYKTTPPVLDSDGSFFLYSKLTVDKSRWQQGNVFSCSVMHEALHNHYTQKSLSLSPGK

SEQ ID NO: 86 - protein, 446 aa, Artificial Sequence
  antibody heavy chain
QVQLQESGPGLVKPSETLSITCTVSGFSLSNYDISWIRQPPGKGLEWLGVIWTGGATNYNPALKSRLTISRDNSKNQVSLKMSSVTAADTAVYYCVRDSNYRYDEPFTYWGQGTLVTVSSASTKGPSVFPLAPCSRSTSESTAALGCLVKDYFPEPVTVSWNSGALTSGVHTFPAVLQSSGLYSLSSVVTVPSSSLGTKTYTCNVDHKPSNTKVDKRVESKYGPPCPPCPAPEAAGGPSVFLFPPKPKDTLMISRTPEVTCVVVDVSQEDPEVQFNWYVDGVEVHNAKTKPREEQFNSTYRVVSVLTVLHQDWLNGKEYKCKVSNKGLPSSIEKTISKAKGQPREPQVYTLPPSQEEMTKNQVSLTCLVKGFYPSDIAVEWESNGQPENNYKTTPPVLDSDGSFFLYSRLTVDKSRWQEGNVFSCSVMHEALHNHYTQKSLSLSLG

SEQ ID NO: 87 - protein, 214 aa, Artificial Sequence
  antibody light chain
EIVLTQSPDTLSVTPKEKVTLTCRASQSIGTNIHWFQQKPGQSPKLLIKYASESISGVPSRFSGSGSGTDFTLTINSVEAEDAATYYCQQSNSWPYTFGQGTKLEIKRTVAAPSVFIFPPSDEQLKSGTASVVCLLNNFYPREAKVQWKVDNALQSGNSQESVTEQDSKDSTYSLSSTLTLSKADYEKHKVYACEVTHQGLSSPVTKSFNRGEC

SEQ ID NO: 88 - protein, 614 aa, Artificial Sequence
  fusion protein
ESKYGPPCPPCPAPEAAGGPSVFLFPPKPKDTLMISRTPEVTCVVVDVSQEDPEVQFNWYVDGVEVHNAKTKPREEQFNSTYRVVSVLTVLHQDWLNGKEYKCKVSNKGLPSSIEKTISKAKGQPREPQVYTLPPSQEEMTKNQVSLTCLVKGFYPSDIAVEWESNGQPENNYKTTPPVLDSDGSFFLYSRLTVDKSRWQEGNVFSCSVMHEALHNHYTQKSLSLSLGGGGGSGGGGSGGGGSQDSTSDLIPAPPLSKVPLQQNFQDNQFHGKWYVVGQAGNIRLREDKDPIKMMATIYELKEDKSYDVTMVKFDDKKCMYDIWTFVPGSQPGEFTLGKIKSFPGHTSSLVRVVSTNYNQHAMVFFKFVFQNREEFYITLYGRTKELTSELKENFIRFSKSLGLPENHIVFPVPIDQCIDGGGGGSGGGGSGGGGSQDSTSDLIPAPPLSKVPLQQNFQDNQFHGKWYVVGQAGNIRLREDKDPIKMMATIYELKEDKSYDVTMVKFDDKKCMYDIWTFVPGSQPGEFTLGKIKSFPGHTSSLVRVVSTNYNQHAMVFFKFVFQNREEFYITLYGRTKELTSELKENFIRFSKSLGLPENHIVFPVPIDQCIDG

SEQ ID NO: 89 - protein, 422 aa, Artificial Sequence
  fusion protein
ESKYGPPCPPCPAPEAAGGPSVFLFPPKPKDTLMISRTPEVTCVVVDVSQEDPEVQFNWYVDGVEVHNAKTKPREEQFNSTYRVVSVLTVLHQDWLNGKEYKCKVSNKGLPSSIEKTISKAKGQPREPQVYTLPPSQEEMTKNQVSLTCLVKGFYPSDIAVEWESNGQPENNYKTTPPVLDSDGSFFLYSRLTVDKSRWQEGNVFSCSVMHEALHNHYTQKSLSLSLGKGGGGSGGGGSGGGGSQDSTSDLIPAPPLSKVPLQQNFQDNQFHGKWYVVGQAGNIRLREDKDPIKMMATIYELKEDKSYDVTMVKFDDKKCMYDIWTFVPGSQPGEFTLGKIKSFPGHTSSLVRVVSTNYNQHAMVFFKFVFQNREEFYITLYGRTKELTSELKENFIRFSKSLGLPENHIVFPVPIDQCIDG

SEQ ID NO: 90 - protein, 639 aa, Artificial Sequence
  fusion protein
QVQLQESGPGLVKPSETLSITCTVSGFSLSNYDISWIRQPPGKGLEWLGVIWTGGATNYNPALKSRLTISRDNSKNQVSLKMSSVTAADTAVYYCVRDSNYRYDEPFTYWGQGTLVTVSSASTKGPSVFPLAPCSRSTSESTAALGCLVKDYFPEPVTVSWNSGALTSGVHTFPAVLQSSGLYSLSSVVTVPSSSLGTKTYTCNVDHKPSNTKVDKRVESKYGPPCPPCPAPEAAGGPSVFLFPPKPKDTLMISRTPEVTCVVVDVSQEDPEVQFNWYVDGVEVHNAKTKPREEQFNSTYRVVSVLTVLHQDWLNGKEYKCKVSNKGLPSSIEKTISKAKGQPREPQVYTLPPSQEEMTKNQVSLTCLVKGFYPSDIAVEWESNGQPENNYKTTPPVLDSDGSFFLYSRLTVDKSRWQEGNVFSCSVMHEALHNHYTQKSLSLSLGGGGGSGGGGSGGGGSQDSTSDLIPAPPLSKVPLQQNFQDNQFHGKWYVVGQAGNIRLREDKDPIKMMATIYELKEDKSYDVTMVKFDDKKCMYDIWTFVPGSQPGEFTLGKIKSFPGHTSSLVRVVSTNYNQHAMVFFKFVFQNREEFYITLYGRTKELTSELKENFIRFSKSLGLPENHIVFPVPIDQCIDG

SEQ ID NO: 91 - protein, 407 aa, Artificial Sequence
  fusion protein
EIVLTQSPDTLSVTPKEKVTLTCRASQSIGTNIHWFQQKPGQSPKLLIKYASESISGVPSRFSGSGSGTDFTLTINSVEAEDAATYYCQQSNSWPYTFGQGTKLEIKRTVAAPSVFIFPPSDEQLKSGTASVVCLLNNFYPREAKVQWKVDNALQSGNSQESVTEQDSKDSTYSLSSTLTLSKADYEKHKVYACEVTHQGLSSPVTKSFNRGECGGGGSGGGGSGGGGSQDSTSDLIPAPPLSKVPLQQNFQDNQFHGKWYVVGQAGNIRLREDKDPIKMMATIYELKEDKSYDVTMVKFDDKKCMYDIWTFVPGSQPGEFTLGKIKSFPGHTSSLVRVVSTNYNQHAMVFFKFVFQNREEFYITLYGRTKELTSELKENFIRFSKSLGLPENHIVFPVPIDQCIDG

SEQ ID NO: 92 - protein, 639 aa, Artificial Sequence
  fusion protein
QDSTSDLIPAPPLSKVPLQQNFQDNQFHGKWYVVGQAGNIRLREDKDPIKMMATIYELKEDKSYDVTMVKFDDKKCMYDIWTFVPGSQPGEFTLGKIKSFPGHTSSLVRVVSTNYNQHAMVFFKFVFQNREEFYITLYGRTKELTSELKENFIRFSKSLGLPENHIVFPVPIDQCIDGGGGGSGGGGSGGGGSQVQLQESGPGLVKPSETLSITCTVSGFSLSNYDISWIRQPPGKGLEWLGVIWTGGATNYNPALKSRLTISRDNSKNQVSLKMSSVTAADTAVYYCVRDSNYRYDEPFTYWGQGTLVTVSSASTKGPSVFPLAPCSRSTSESTAALGCLVKDYFPEPVTVSWNSGALTSGVHTFPAVLQSSGLYSLSSVVTVPSSSLGTKTYTCNVDHKPSNTKVDKRVESKYGPPCPPCPAPEAAGGPSVFLFPPKPKDTLMISRTPEVTCVVVDVSQEDPEVQFNWYVDGVEVHNAKTKPREEQFNSTYRVVSVLTVLHQDWLNGKEYKCKVSNKGLPSSIEKTISKAKGQPREPQVYTLPPSQEEMTKNQVSLTCLVKGFYPSDIAVEWESNGQPENNYKTTPPVLDSDGSFFLYSRLTVDKSRWQEGNVFSCSVMHEALHNHYTQKSLSLSLG

SEQ ID NO: 93 - protein, 407 aa, Artificial Sequence
  fusion protein
QDSTSDLIPAPPLSKVPLQQNFQDNQFHGKWYVVGQAGNIRLREDKDPIKMMATIYELKEDKSYDVTMVKFDDKKCMYDIWTFVPGSQPGEFTLGKIKSFPGHTSSLVRVVSTNYNQHAMVFFKFVFQNREEFYITLYGRTKELTSELKENFIRFSKSLGLPENHIVFPVPIDQCIDGGGGGSGGGGSGGGGSEIVLTQSPDTLSVTPKEKVTLTCRASQSIGTNIHWFQQKPGQSPKLLIKYASESISGVPSRFSGSGSGTDFTLTINSVEAEDAATYYCQQSNSWPYTFGQGTKLEIKRTVAAPSVFIFPPSDEQLKSGTASVVCLLNNFYPREAKVQWKVDNALQSGNSQESVTEQDSKDSTYSLSSTLTLSKADYEKHKVYACEVTHQGLSSPVTKSFNRGEC

SEQ ID NO: 94 - protein, 832 aa, Artificial Sequence
  fusion protein
QVQLQESGPGLVKPSETLSITCTVSGFSLSNYDISWIRQPPGKGLEWLGVIWTGGATNYNPALKSRLTISRDNSKNQVSLKMSSVTAADTAVYYCVRDSNYRYDEPFTYWGQGTLVTVSSASTKGPSVFPLAPCSRSTSESTAALGCLVKDYFPEPVTVSWNSGALTSGVHTFPAVLQSSGLYSLSSVVTVPSSSLGTKTYTCNVDHKPSNTKVDKRVESKYGPPCPPCPAPEAAGGPSVFLFPPKPKDTLMISRTPEVTCVVVDVSQEDPEVQFNWYVDGVEVHNAKTKPREEQFNSTYRVVSVLTVLHQDWLNGKEYKCKVSNKGLPSSIEKTISKAKGQPREPQVYTLPPSQEEMTKNQVSLTCLVKGFYPSDIAVEWESNGQPENNYKTTPPVLDSDGSFFLYSRLTVDKSRWQEGNVFSCSVMHEALHNHYTQKSLSLSLGGGGGSGGGGSGGGGSQDSTSDLIPAPPLSKVPLQQNFQDNQFHGKWYVVGQAGNIRLREDKDPIKMMATIYELKEDKSYDVTMVKFDDKKCMYDIWTFVPGSQPGEFTLGKIKSFPGHTSSLVRVVSTNYNQHAMVFFKFVFQNREEFYITLYGRTKELTSELKENFIRFSKSLGLPENHIVFPVPIDQCIDGGGGGSGGGGSGGGGSQDSTSDLIPAPPLSKVPLQQNFQDNQFHGKWYVVGQAGNIRLREDKDPIKMMATIYELKEDKSYDVTMVKFDDKKCMYDIWTFVPGSQPGEFTLGKIKSFPGHTSSLVRVVSTNYNQHAMVFFKFVFQNREEFYITLYGRTKELTSELKENFIRFSKSLGLPENHIVFPVPIDQCIDG

SEQ ID NO: 95 - DNA, 474 bp, Homo sapiens
catcatctgctggcctctgacgaagagatccaggatgtgtccggcacctggtatctgaaggccatgaccgtggaccgcgagttccctgagatgaacctggaaagcgtgacccctatgacactgaccacactggaaggcggcaacctggaagccaaagtgaccatgctgatctccggccggtgccaagaagtgaaggccgtcctggaaaagaccgacgagcctggcaagtacaccgctgatggcggcaagcacgtggcctacatcatcagatcccacgtgaaggaccactacatcttctactgcgagggcgagctgcacggaaagcctgttagaggcgtgaagctcgtgggcagagatcccaagaacaatctggaagccctggaagatttcgagaaggccgctggcgctagaggcctgtccacagagtctatcctgattcctcggcagtccgagacatgctcccctggctctgat

SEQ ID NO: 96 - DNA, 534 bp, Homo sapiens
caggatagcaccagcgatctgattccggcgccgccgctgagcaaagtgccgctgcagcagaactttcaggataaccagtttcagggcaaatggtatgtggtgggcctggcgggcaacgcgattctgcgcgaagataaagatccgcagaaaatgtatgcgaccatttatgaactgaaagaagataaaagctataacgtgaccagcgtgctgtttcgcaaaaaaaaatgcgattattggattcgcacctttgtgccgggctgccagccgggcgaatttaccctgggcaacattaaaagctatccgggcctgaccagctatctggtgcgcgtggtgagcaccaactataaccagcatgcgatggtgttttttaaaaaagtgagccagaaccgcgaatattttaaaattaccctgtatggccgcaccaaagaactgaccagcgaactgaaagaaaactttattcgctttagcaaaagcctgggcctgccggaaaaccatattgtgtttccggtgccgattgatcagtgcattgatggc

SEQ ID NO: 97 - DNA, 534 bp, Artificial Sequence
  lipocalin mutein
caggatagcaccagcgatctgattccggcgccgccgctgagcaaagtgccgctgcagcagaactttcaggataaccagtttcatggcaaatggtatgtggtgggcctggcgggcaacgcgattctgcgcgaagataaagatccgcagaaaatgtatgcgaccatttatgaactgaaagaagataaaagctataacgtgaccagcgtgctgtttcgcaaaaaaaaatgcgattattggattcgcacctttgtgccgggcagccagccgggcgaatttaccctgggcaacattaaaagctatccgggcctgaccagctatctggtgcgcgtggtgagcaccaactataaccagcatgcgatggtgttttttaaaaaagtgagccagaaccgcgaatattttaaaattaccctgtatggccgcaccaaagaactgaccagcgaactgaaagaaaactttattcgctttagcaaaagcctgggcctgccggaaaaccatattgtgtttccggtgccgattgatcagtgcattgatggc

SEQ ID NO: 98 - DNA, 534 bp, Artificial Sequence; identical to SEQ ID NO: 97
  lipocalin mutein

SEQ ID NO: 99 - DNA, 456 bp, Artificial Sequence
  lipocalin mutein
gcctcagacgaggagattcaggatgtgtcagggacgtggtatctgaaggccatgacggtggatgaggggtgtcgtccttggaatatattttcagttacgccaatgactctgactacccttgaaggcggcaatctggaggctaaggtcaccatggcaatagatgggccggcacaggaggtgaaagcagtgttagagaagacagatgaaccgggtaaatatacggccgatggcggtaaacatgttgcctatatcattcgcagccatgtgaaagatcattacatcttttatagcgagggcgtgtgcgatgggtctcctgttccaggggtgtggctcgtgggcagagaccccaagaacaacctggaagccttggaggactttgagaaagccgcaggagcccgcggactcagcacggagagcatcctcatccccaggcagagcgaaaccagctctccaggg

SEQ ID NO: 100 - DNA, 456 bp, Artificial Sequence
  lipocalin mutein
acctcagacgaggagattcaggatgtgtcagggacgtggtatctgaaggcgatgacggtggatgaggggtgtcgtccttggaatatattttcagttacgccaatgactctgactacccttgaaggcggcaatctggaggctaaggtcaccatggcaatagatgggccggcacaggaggtgagagcagtgttagagaagacagatgaaccgggtaaatatacggccgacggcggtaaacatgatgcctatatcattcgcagccatgtgaaagatcattacatcttttatagcgagggcgtgtgcgatgggtctcctgttccgggggtgtggctcgtgggcagagaccccgagaacaacctggaagccttggaggactttgagaaaaccgcaggagcccgcggactcagcacggagagcatcctcatccccaggcagagcgaaaccagctctccaggg

SEQ ID NO: 101 - DNA, 456 bp, Artificial Sequence
  lipocalin mutein
gcctcagacgaggagattcaggatgtgtcagggacgtggtatctgaaggcgatgacggtggatgaggggtgtcgtccttggaatatattttcagttacgccaatgactctgactacccttgaaggcggcaatctggaggctaaggtcaccatggcaatagatgggccggcacaggaggtgaacgcagtgttagagaagacagatgaaccgggtaaatatacggccgatggcggtaaacatgttgcctatatcattcgcagccatgtgagagatcattacatcttttatagcgagggcgtgtgcgatgggtctcctgttccgggggtgtggctcgtgggcagggaccccgagaacaacctggaagccttggaggactttgagaaaaccgcaggagcccgcggactcagcacggagagcattctcattcccaggcagagcgaaaccagctctccaggg

SEQ ID NO: 102 - DNA, 456 bp, Artificial Sequence
  lipocalin mutein
gtctcagacgaggagattcaggatgtgtcagggacgtggtatctgaaggcgatgacggtggatgaggggtgtcgtccttggaatatattttcagttacgccaatgactctgactacccttgaaggcggcaatctggaggctaaggtcaccatggcaatagatgggccggcacaggaggtgagagcagtgttagagaagacagatgaaccgggtaaatatacggccgatggcggtaaacatgttgcctatatcattcgcagccatgtggaagatcattacatcttttatagcgagggcgtgtgcgatgggtctcctgttccgggggtgtggctcgtgggcagagaccccgagaacaacctggaagccttggaggactttgagaaaaccgcaggagcccgcggactcagcacggagagcatcctcatccccaggcagagcgaaaccagctctccaggg

SEQ ID NO: 103 - DNA, 456 bp, Artificial Sequence
  lipocalin mutein
gcctcagacgaggagattcaggatgtgtcagggacgtggtatctgaaggcgatgacggtggatgaggggtgtcgtccttggaatatattttcagttacgccaatgactctgtctacccttgaaggcggcaatctggaggctaaggtcaccatggcaatagatgggccggcacaggaggtgaaagcagtgttagagaagacagatgaaccgggtaaatatacggccgatggcggtaaacatgttgcctatatcattcgcagccatgtgaaagatcattacatcttttatagcgagggcgtgtgcgatgggtctcctgttccgggggtgtggctcgtgggcagagaccccaagaacaacctggaagccttggaggactttgagaaagccgcaggagcccgcggactcagcacggagagcatcctcatccccaggcagatcgaaaccagctctccaggg

SEQ ID NO: 104 - DNA, 456 bp, Artificial Sequence
  lipocalin mutein
gcctcagacgaggagattcaggatgtgtcagggacgtggtatctgaaggcgatgacggtggatgaggggtgtcgtccttggaatatattttcagttacgccaatgactctgactacccttgaaggcggcaatctggaggctgaggtcaccatggcaatagatgggccggcacaggaggtgaaagcagtgttagagaaggcagatgaaccgggtaaatatacggccgatggcggtaaacatgttgcctatatcattcgcagccatgtgaaagatcattacatcttttatagcgagggcgtgtgcgatgggtctcctgttccgggggtgtggctcgtgggcagagaccccaagaacaacctggaagccttggaggactttgagaaaaccgcaggagcccgcggactcagcacggagagcatcctcatccccagtcagatcgaaaccagctctccaggg

SEQ ID NO: 105 - DNA, 456 bp, Artificial Sequence
  lipocalin mutein
acctcagacgaggagattcaggatgtgtcagggacgtggtatctgaaggcgatgacggtggatgaggggtgtcgtccttggaatatattttcagttacgccaatgactctgactacccttgaagacggcaatctggaggctaaggtcaccatggcaatagatgggccggcacaggaggtgaaagcagtgttagagaaggcagatgaaccgggtaaatatacggccgatggcggtaaacatgttgcctatatcattcgcagccatgtgaaagatcattacatcttttatagcgagggcgtgtgcgatgggtctcctgttccgggggtgtggctcgtgggcagagaccccaagaacaacctggaagccttggaggactttgagaaagccgcaggagcccgcggactcagcacggagagcatcctcatccccaggcagatcgaaaccagctctccaggg

SEQ ID NO: 106 - DNA, 534 bp, Artificial Sequence
  lipocalin mutein
caggactccacctcagacctgatcccagccccacctctgagcaaggtccctctgcagcagaacttccaggacaaccaattccatgggaagtggtatgtggtaggtcaggcagggaatatcaaactcagagaagacaaagacccgaacaagatgatggccaccatctatgagctgaaagaagacaagagctacaatgtcaccggtgtcacttttgacgacaagaagtgtacttacgctatctctacttttgttccaggttcccagccaggcgagttcacgctgggcaaaattaagagtttccctggacatacgagttctctcgtccgagtggtgagcaccaactacaaccagcatgctatggtgttcttcaagttcgttttccaaaacagggaggaattctacatcaccctctacgggagaaccaaggagctgacttcggaactaaaggagaacttcatccgcttctccaaatctctgggcctccctgaaaaccacatcgtcttccctgtcccaatcgaccagtgtatcgacggc

SEQ ID NO: 107 - DNA, 534 bp, Artificial Sequence
  lipocalin mutein
caggactccacctcagacctgatcccagccccacctctgagcaaggtccctctgcagcagaacttccaggacaaccaattccatgggaaatggtacgttgtcgggcaggccggaaatattaggctgcgtgaggataaggatccgattaaaatgatggcgaccatttacgagttgaaagaagataaatcatatgacgtcaccatggtgaagtttgatgataagaaatgcatgtacgatatttggacctttgtgccggggagccagccgggcgagtttactttaggcaagattaaaagttttccgggccatacatcatcgttggtccgcgtcgtgagcaccaactacaaccagcatgccatggtgttcttcaagtttgtgtttcagaaccgcgaggagttttatatcacactgtacgggcgcacgaaagaactgacaagcgagctgaaggaaaattttatccgcttttccaaatctctgggcctccctgaaaaccacatcgtcttccctgtcccaatcgaccagtgtatcgacggc

SEQ ID NO: 108 - DNA, 534 bp, Artificial Sequence
  lipocalin mutein
caggactccacctcagacctgatcccagccccacctctgagcaaggtccctctgcagcagaacttccaggacaaccaattccatgggaaatggtacgttgtcgggcaggccggaaatattaggctgcgtgaggataaggatccgaataaaatgatggcgaccatttacgagttgaaagaagataaatcatatgacgtcaccgcggtggcgtttgatgataagaaatgcacgtacgatatttggacctttgtgccggggagccagccgggcgagtttactttaggcaagattaaaagttttccgggccatacatcatcgttggtccgcgtcgtgagcaccaactacaaccagcatgccatggtgttcttcaagtttgtgtttcagaaccgcgaggagttttatatcacactgtacgggcgcacgaaagaactgacaagcgagctgaaggaaaattttatccgcttttccaaatctctgggcctccctgaaaaccacatcgtcttccctgtcccaatcgaccagtgtatcgacggc

SEQ ID NO: 109 - DNA, 534 bp, Artificial Sequence
  lipocalin mutein
caggactccacctcagacctgatcccagccccacctctgagcaaggtccctctgcagcagaacttccaggacaaccaattccatgggaaatggtacgttgtcgggcaggccggaaatattaagctgcgtgaggataaggatccgaataaaatgatggcgaccatttacgagttgaaagaagataaatcatatgacgtcaccgcggtggcgtttgatgataagaaatgcacgtacgatatttggacctttgtgccggggagccagccgggcgagtttactttaggcaagattaaaagttttccgggccatacatcatctttggtccgcgtcgtgagcaccaactacaaccagcatgccatggtgttcttcaagtttgtgtttcagaaccgcgaggagttttatatcacactgtacgggcgcacgaaagaactgacaagcgagctgaaggaaaattttatccgcttttccaaatctctgggcctccctgaaaaccacatcgtcttccctgtcccaatcgaccagtgtatcgacggc

SEQ ID NO: 110 - DNA, 525 bp, Artificial Sequence
  lipocalin mutein
caggactccacctcagacctgatcccagccccacctctgagcaaggtccctctgcagcagaacttccaggacaaccaattccatgggaaatggtacgttgtcgggcaggccggaaatattaagctgcgtgaggatagtaaaatgatggcgaccatttacgagttgaaagaagataaatcatatgacgtcaccggtgtgagttttgatgataagaaatgcacgtacgctattatgacctttgtgccggggagccagccgggcgagtttactttaggcaagattaaaagttttccgggccatacatcatcgttggtccgcgtcgtgagcaccaactacaaccagcatgccatggtgttcttcaagtttgtgtttcagaaccgcgaggagttttatatcacactgtacgggcgcacgaaagaactgacaagcgagctgaaggaaaattttatccgcttttccaaatctctgggcctccctgaaaaccacatcgtcttccctgtcccaatcgaccagtgtatcgacggc

SEQ ID NO: 111 - DNA, 534 bp, Artificial Sequence
  lipocalin mutein
caggactccacctcagacctgatcccagccccacctctgagcaaggtccctctgcagcagaacttccaggacaaccaattccatgggaaatggtacgttgtcgggcaggccggaaatattaagctgcgtgaggataaggatccggttaaaatgatggcgaccatttacgagttgaaagaagataaatcatatgacgtcaccggggtgacgtttgatgataagaaatgcaggtacgatatttcgacctttgtgccggggagccagccgggcgagtttacttttggcaagattaaaagttttccgggccatacatcatcgttggtccgcgtcgtgagcaccaactacaaccagcatgccatggtgttcttcaagtttgtgtttcagaaccgcgaggagttttatatcacactgtacgggcgcacgaaagaactgacaagcgagctgaaggaaaattttatccgcttttccaaatctctgggcctccctgaaaaccacatcgtcttccctgtcccaatcgaccagtgtatcgacggc

SEQ ID NO: 112 - DNA, 534 bp, Artificial Sequence
  lipocalin mutein
caggactccacctcagacctgatcccagccccacctctgagcaaggtccctctgcagcagaacttccaggacaaccaattccatgggaaatggtacgttgtcgggcaggccggaaatattaggctgcgtgaggataaggatccgcataaaatgatggcgaccatttacgagttgaaagaagataaatcatatgacgtcaccggggtgacttttgatgataagaaatgcacgtacgctatttcgacctttgtgccggggagccagccgggcgagtttactttaggcaagattaaaagttttccgggccatacatcatctttggtccgcgtcgtgagcaccaactacaaccagcatgccatggtgttcttcaagtttgtgtttcagaaccgcgaggagttttatatcacactgtacgggcgcacgaaagaactgacaagcgagctgaaggaaaattttatccgcttttccaaatctctgggcctccctgaaaaccacatcgtcttccctgtcccaatcgaccagtgtatcgacggc

SEQ ID NO: 113 - DNA, 534 bp, Artificial Sequence
  lipocalin mutein
caggactccacctcagacctgatcccagccccacctctgagcaaggtccctctgcagcagaacttccaggacaaccaattccatgggaaatggtacgttgtcgggcaggccggaaatattaagctgcgtgaggataaggatccgaataaaatgatggcgaccatttacgagttgaaagaagataaatcatatgacgtcaccggggtgacttttgatgataagaaatgcacgtacgctatttctacccttgtgccggggagccagccgggcgagtttacttttggcaagattaaaagttttccgggccatacatcatcgttggtccgcgtcgtgagcaccaactacaaccagcatgccatggtgttcttcaagtttgtgtttcagaaccgcgaggagttttatatcacactgtacgggcgcacgaaagaactgacaagcgagctgaaggaaaattttatccgcttttccaaatctctgggcctccctgaaaaccacatcgtcttccctgtcccaatcgaccagtgtatcgacggc

SEQ ID NO: 114 - DNA, 534 bp, Artificial Sequence
  lipocalin mutein
caggactccacctcagacctgatcccagccccacctctgagcaaggtccctctgcagcagaacttccaggacaaccaattccatgggaaatggtacgttgtcgggcaggccggaaatattaggctgcgtgaggataaggatccgtctaaaatgatggcgaccatttacgagttgaaagaagataaatcatatgacgtcaccgctgtgacgtttgatgataagaaatgcaattacgctatttctacctttgtgccggggagccagccgggcgagtttactttaggcaagattaaaagttttccgggccatacatcatcgttggtccgcgtcgtgagcaccaactacaaccagcatgccatggtgttcttcaagtttgtgtttcagaaccgcgaggagttttatatcacactgtacgggcgcacgaaagaactgacaagcgagctgaaggaaaattttatccgcttttccaaatctctgggcctccctgaaaaccacatcgtcttccctgtcccaatcgaccagtgtatcgacggc

SEQ ID NO: 115 - DNA, 534 bp, Artificial Sequence
  lipocalin mutein
caggactccacctcagacctgatcccagccccacctctgagcaaggtccctctgcagcagaacttccaggacaaccaattccatgggaaatggtatgtcgtgggcatggccggaaataatctgctgcgtgaggataaggatccgcacaaaatgagcgcgaccatttacgagttgaaagaagataaatcatataacgtcaccgacgtgatgtttctggacaagaaatgccaatacatcatttggacctttgtgccggggagccagccgggcgagtttactttaggcttcattaaaagtgacccgggccacacatcatacttggtccgcgtcgtgagcaccaactacaaccagcatgccatggtgttcttcaagagcgtgatccagaaccgcgagtggtttggaatcacactgtacgggcgcacgaaagaactgacaagcgagctgaaggaaaattttatccgcttttccaaatctctgggcctccctgaaaaccacatcgtcttccctgtcccaatcgaccagtgtatcgacggc

SEQ ID NO: 116 - DNA, 535 bp, Artificial Sequence
  lipocalin mutein
caggactccacctcagacctgatcccagccccacctctgagcaaggtccctctgcagcagaacttccaggacaaccaattccaagggaaatggtatgtcgtgggcatggccggaaataatctgctgcgtgaggataaggatccgcacaaaatgagcgcgaccatttacgagttgaaagaagataaatcatataacgtcaccgacgtgatgtttctggacaagaaatgccaatacatcatttggacctttgtgccggggagccagccgggcgagcttactttaggcttcattagaagtgacctgggccacacatcatacttggtccgcgtcgtgagcaccaactacaaccagcatgccatggtgttcttcaagagcgtgatccagaaccgcgagtggtttggaatcacactgtacgggcgcacgaaagaactgacaagcgagctgaaggaaaattttatccgcttttccaaatctctgggcctccctgaaaaccacatcgtcttccctgtcccaatcgaccagtgtatcgacggca

SEQ ID NO: 117 - DNA, 535 bp, Artificial Sequence
  lipocalin mutein
caggactccacctcagacctgatccctgccccacctctgagcaaggtccctctgcagcagaacttccaggactaccaattccaagggaaatggtatgtcgtgggcatggccggaaataatctgctgcgtgaggataaggatccgcacaaaatgggcgcgaccatttacgagttgaaagaagataaatcatataacgtcaccgacgtgatgcttctggacaagaaatgccaatacatcattcagacctttgtgccggggagccagccgggcgagtctactttaggcttcattaaaagtgacccgggccacacatcatacttggtccgcgtcgtgagcaccaactacaaccagcatgccatggtgttcttcaagagcgtgatccagaaccgcgagtggtttggaatcacactgtacgggcgcacgaaagaactgacaagcgagctgaaggaaaattttatccgcttttccaaatctctgggcctccctgaaaaccacatcgtcttccctgtcccaatcgaccagtgtatcgacggca

SEQ ID NO: 118 - DNA, 535 bp, Artificial Sequence
  lipocalin mutein
caggactccacctcagacctgatcccagccccacctctgagcaaggtccctctgcagcagaacttccaggacaaccaattccaagggaaatggtatgtcgtgggcatggccggaaataatctgctgcgtgaggataaggatccgcacaaaatgggcgcgaccatttacgagttgaaagaagataaatcatataacgtcaccgacgtgatgtttctggacaagaaatgccaacacatcatatggacctttgtgccggggagccagccgggcgagttaactttaggcttcattaaaagtgacccgggccacacatcatacttggtccgcgtcgtgagcaccaactacaaccagcatgccatggtgttcttcaagagcgtgatccagaaccgcgagtggtttggaatcacactgtacgggcgcacgaaagaactgacaagcgagctgaaggaaaattttatccgcttttccaaatctctgggcctccctgaaaaccacatcgtcttccctgtcccaatcgaccagtgtatcgacggca

SEQ ID NO: 119 - DNA, 535 bp, Artificial Sequence
  lipocalin mutein
caggactccacctcagacctgatcccagccccacctctgagcaaggtccctctgcagcagaacttccaggacgaccaattccaagggaaatggtatgtcgtgggcatggccggaaataatctgttgcgtgaggataaggatccgcacaaaatgggcgcgaccatttacgagttgaaagaagataaatcatataacgtcaccgacgtgatgtttctggacaagaaatgccaatacatcatttggacctttgtgccggggagccagccgggcgagttgactttaggcttcattaaaagtgacccgggccacacatcatacttggtccgcgtcgtgagcaccaactacaaccagcatgccatggtgttcttcaagagcgtgatccagaaccgcgagtggtttggaatcacactgtacgggcgcacgaaagaactgacaagcgagctgaaggaaaattttatccgcttttccaaatctctgggcctccctgaaaaccacatcgtcttccctgtcccaatcgaccagtgtatcgacggca

SEQ ID NO: 120 - DNA, 535 bp, Artificial Sequence
  lipocalin mutein
caggactccacctcagacctgatcccagccccacctctgagcaaggtccctctgcagcagaacttccaggacaaccaattccaagggaaatggtatatcgtgggcatggccggaaataatctgctgcgtgaggataaggatccgcacaaaatgggcgcgaccatttacgagttgaaagaagataaatcatataacgtcaccgacgtgatgtttctggacaagaaatgccaatacatcatttggacctttgtgccggggagccagccgggcgagcttactttaggcttcattaaaagtgacccgggccacacatcatacttggtccgcgtcgtgagcaccaactacaaccagcatgccatggtgttcttcaagagcgtgatccagaaccgcgagtggtttggaatcacactgtacgggcgcacgaaagaactgacaagcgagctgaaggaaaattttatccgcttttccaaatctctgggcctccctgaaaaccacatcgtcttccctgtcccaatcgaccagtgtatcgacggca

SEQ ID NO: 121 - DNA, 535 bp, Artificial Sequence
  lipocalin mutein
caggactccacctcagacctgatcccagccccacctctgagcaaggtccctctgcagcggaacttccaggacaaccaattccaagggaagtggtatgtcgtgggcatggccggaaataatctgctgcgtgtggataaggatccgcacaaaatgggcgcgaccatttacgagttgaaagaagataaatcatataacgtcaccgacgtgatgtttctggacaagaaatgccaatacatcatttggacctttgtgccggggagccagccgggcgagttaactttaggcttcattaaaagtgacccgggccacacatcatacttggtccgcgtcgtgagcaccaactacaaccagcatgccatggtgtacttcaagagcgtgatccagaaccgcgagtggtttggaatcacactgtacgggcgcacgaaagaactgacaagcgagctgaaggaaaattttatccgcttttccaaatctctgggcctccctgaaaaccacatcgtcttccctgtcccaatcgaccagtgtatcgacggca

SEQ ID NO: 122 - DNA, 535 bp, Artificial Sequence
  lipocalin mutein
caggactccacctcagatctgatcccagccccacctctgagcaaggtccctctgcagcagaacttccaggacaaccaattccaagggaaatggtatgtcgtgggcatggccggaaataatctgctgcgtgaggataaggatccgcacaaaatgagcgcgaccatttacgagttgaaagaagataaatcatataacgtcaccgacgtgatgtttctggacaagaaatgccaatacatcaattggccctttgtgccggggagccagccgggcgagtttactttaggcttcattaaaagtgacctgggccccacatcatacttggtccgcgtcgtgagcaccaactacaaccagcatgccatggtgttcttcaagagcgtgatccagaaccgcgagtggtttggaatcacactgtacgggcgcacgaaagaactgacaagcgagctgaaggaaaattttatccgcttttccaaatctctgggcctccctgaaaaccacatcgtcttccctgtcccaatcgaccagtgtatcgacggca

SEQ ID NO: 123 - DNA, 535 bp, Artificial Sequence
  lipocalin mutein
caggactccacctcagacctgatcccagccccacctctgagcaaggtccctctgcagcagaacttccaggacaaccaattccaagggaaatggtatgtcgtgggcatggccggaaataatctgctgcgtgaggataaggatccgcacaaaatgggtgcgaccatttacgagttgaatgaagataaatcatataacgtcaccgacgtgatgtttctggacaagaaatgccaatacatcatttggacctttgtgccggggagccagccgggcgagcttactttaggcttcattaaaagtgacccgggccacacatcatacttggtccgcgtcgtgagcaccaactacaaccagcatgccatggtgttcttcaagagcgtgatccagaaccgcgagtggtttggaatcacactgtacgggcgcacgaaagaactgacaagcgagctgaaggaaaattttatccgcttttccaaatctctgggcctccctgaaaaccacatcgtcttccctgtcccaatcgaccagtgtatcgacggca

SEQ ID NO: 124 - DNA, 535 bp, Artificial Sequence
  lipocalin mutein
caggactccacctcagacctgatcccagccccacctctgagcaaggtccctctgcagcagaacttccaggacaaccaattccaagggaaatggtatgtcgtgggcatggccggaaataatctgctgcgtgatgataaggatccgcacaaaatgagcgctaccatttacgagttgaaagaagataaatcatataacgtcaccgacgtgatgttactggacaagaaatgccattacatcatttggacctttgtgccggggagccagccgggcgagcttactttaggcttcattaaaagtgacccgggccacacatcatacttggtccgcgtcgtgagcaccaactacaaccagcatgccatggtgttcttcaaaagcgtgatccagaaccgcgagtggtttggaatcacactgtacgggcgcacgaaagaactgacaagcgagctgaaggaaaattttatccgcttttccaaatctctgggcctccctgaaaaccacatcgtcttccctgtcccaatcgaccagtgtatcgacggca

SEQ ID NO: 125 - DNA, 360 bp, Artificial Sequence
  antibody heavy chain variable region
caggtgcaactgaaggagtcaggacctggcctggtggcgccctcacagaacctgtccattacctgcactgtctctgggttctcattaagcaactatgatataagctggattcgccagccaccaggaaagggtctggagtggctcggagtaatatggactggtggagccacaaattataattcagctttcatgtccagactgagcatcagtagggacaactccaagagccaagttttcttaaaaatgaacagtctgcaaactgatgacacagccatatattactgtgtgagagattcgaactataggtacgacgagccgtttacttactggggccaagggactctggtcactgtctctgca

SEQ ID NO: 126 - DNA, 360 bp, Artificial Sequence
  antibody heavy chain variable region
caggtccagctgcaggagtcaggccccggcctggtgaagcccagtgagaacctgtcaatcacctgcacagtctctggcttctcactgagcaattacgacatcagttggattcgacagccccctggaaagggcctggaatggctgggcgtgatctggacaggcggggcaactaactataatccagcctttaaaagccggctgaccatttccagagacaactccaagtctcaggtgtctctgaaaatgagctccctgcaggccgctgataccgctgtgtactattgtgtcagggacagcaattaccgctatgatgagcccttcacatactgggggcagggaactctggtgaccgtctctagt

SEQ ID NO: 127 - DNA, 360 bp, Artificial Sequence
  antibody heavy chain variable region
caggtccagctgcaggagtccggccccggcctggtgaagccctccgagacactgtctatcacctgcacagtcagcggcttctcactgagcaactacgacatctcctggattcgacagccccctggaaagggcctggaatggctgggcgtgatctggacaggcggggcaactaactataatccagccctgaaatctcggctgactattagtagagacaactcaaagaatcaggtgtccctgaaaatgagctccgtcaccgccgctgatacagctgtgtactattgtgtcagggacagcaattaccgctatgatgagccctttacctactgggggcagggaactctggtgaccgtctctagt

SEQ ID NO: 128 - DNA, 351 bp, Artificial Sequence
  antibody heavy chain variable region
gaggttcagctgcagcagtctggggcagagcttgtgaagccaggggcctcagtcaagttgtcctgcacagcttctggcttcgacattaaagacacctatatccactgggtgaagcagaggcctgaacagggcctggagtggattggaaggattgatcctgcggacggtaatactaggtatgacccgaagttccaggacaagaccactataacaaccgacacatcctccaacacagcccacctgcagctcagcagcctgacatctgaggacactgccgtctattactgtgctagaggcctcggagcttggtttgcttcctggggccaagggactctggtcactgtctctgca

SEQ ID NO: 129 - DNA, 372 bp, Artificial Sequence
  antibody heavy chain variable region
gaggttcagctgcagcagtctggggcagagcttgtgaagccaggggcctcagtcaagttgtcctgcacagcttctggcttcaacattaaagacacctatatgtactgggtgaagcagaggcctgaacagggcctggagtggattggaaggattgatcctgcgaatggtaatactaaatatgacccgaagttccagggcaaggccactataacagcagacacatccgccaacacagcctacctgcagctcagcagcctgacatctgaggacactgccgtctattactgttctagaggccctccaggaggtatcggcgagtatatctatgctatggactactggggtcaaggaacctcagtcaccgtctcctca

SEQ ID NO: 130 - DNA, 318 bp, Artificial Sequence
  antibody light chain variable region
gacatcttgctgactcagtctccagccatcctgtctgtgagtccaggagaaagagtcagtctctcctgcagggccagtcagagcattggcacaaacatacactggtttcagcaaagaacaaatggttctccaaggcttctcataaagtatgcttctgagtctatctctgggatcccttccaggtttagtggcagtggatcagggacagattttactcttagcatcaacagtgtggagtctgaagatattgcagattactactgtcaacaaagtaatagctggccgtacacgttcggaggggggaccaagctggaaata

SEQ ID NO: 131 - DNA, 321 bp, Artificial Sequence
  antibody light chain variable region
gaaatcgtgctgacacagagccctgacacactgagcgtgactcccaaggagaaagtcaccctgacatgccgggcatcacagagcatcggaacaaacattcactggttccagcagagaccaggccagagccccaagctgctgatcaaatacgcctccgaatctatcagtggcattccttcccgattctcaggcagcgggtccggaaccgactttactctgaccattaactctgtggaggctgaagatgccgctacatactattgccagcagtctaatagttggccttataccttcggccaggggacaaagctggagatcaaa

SEQ ID NO: 132 - DNA, 321 bp, Artificial Sequence
  antibody light chain variable region
gaaatcgtgctgacacagtctcctgataccctgagcgtgactcccaaggagaaagtcaccctgacatgcagggcatcacagagcatcggaacaaacattcactggttccagcagaagccaggccagagccccaagctgctgatcaaatacgcctccgaatctattagtggagtgccttcccgcttctcaggcagcgggtccggaaccgactttactctgaccatcaactctgtggaggctgaagatgccgctacatactattgccagcagtctaatagttggccttataccttcggccaggggacaaagctggagatcaaa

SEQ ID NO: 133 - DNA, 318 bp, Artificial Sequence
  antibody light chain variable region
gatatccagatgacacagactacatcctccctgtctgcctctctgggagacagagtcaccatcagttgcagggcaagtcaggacattaccaattccttaaactggtatcagcagaaaccagatggaactgttaaactcctgatccactacacatcaagattacactcaggagtcccatcaaggttcagtggcagtgggtctggaacagattattctctcaccattagcaacctggagcaagaagatattgccacttacttttgccaacagggtcatacgcttcctccgacgttcggtggaggcaccaagctggaaatc

SEQ ID NO: 134 - DNA, 321 bp, Artificial Sequence
  antibody light chain variable region
caaattgttctcacccagtctccagcaatcatgtctgcatctctaggggaacgggtcaccatgacctgcactgccagctcaagtgtaagttccagttacttgcactggtaccagcagaagccaggatcctcccccaaactctggatttatagcacatccaacctggcttctggagtcccagctcgcttcagtggcagtgggtctgggacctcttactctctcacaatcagcagcatggaggctgaagatgctgccacttattactgccaccagtatcatcgttccccacccacgttcggtggaggcaccaagctggaaatc

SEQ ID NO: 135 - DNA, 1350 bp, Artificial Sequence
  antibody heavy chain
caggtccagctgcaagagtctggccctggactggtcaagccttccgagacactgtccatcacctgtaccgtgtccggcttctccctgtccaactacgacatctcctggatcagacagcctcctggcaaaggcctggaatggctgggagtgatttggaccggcggagccaccaactacaaccccgctctgaagtcccggctgaccatctccagagacaactccaagaaccaggtgtccctgaagatgtcctccgtgaccgctgctgataccgccgtgtactactgcgtgcgggactccaactacagatacgacgagcccttcacctactggggccagggaacactggtcaccgtgtcctctgcttccaccaagggaccctctgtgttccctctggctccttccagcaagtctacctctggcggaacagctgctctgggctgcctggtcaaggactactttcctgagccagtgaccgtgtcttggaactctggcgctctgacatccggcgtgcacacctttccagctgtgctgcaatcctccggcctgtactctctgtccagcgtcgtgaccgtgccttctagctctctgggcacccagacctacatctgcaatgtgaaccacaagcctagcaacaccaaggtggacaagaaggtggaacccaagtcctgcgacaagacccacacctgtcctccatgtcctgctccagaagctgctggcgccccttccgtgtttctgttccctccaaagcctaaggacaccctgatgatctctcggacccctgaagtgacctgcgtggtggtggatgtgtctcacgaggatcccgaagtgaagttcaattggtacgtggacggcgtggaagtgcacaacgccaagaccaagcctagagaggaacagtacaacagcacctacagagtggtgtccgtgctgaccgtgctgcaccaggattggctgaacggcaaagagtacaagtgcaaggtgtccaacaaggccctgcctgctcctatcgaaaagaccatcagcaaggccaagggccagcctagggaaccccaggtttacaccttgcctccatctcgggacgagctgacaaaaaatcaggtttccctgacctgcctcgtgaagggattctacccctccgatatcgccgtggaatgggagtctaatggccagcctgagaacaactacaagacaacccctcctgtgctggactccgacggctcattcttcctgtactccaagctgacagtggacaagtccagatggcagcagggcaacgtgttctcctgctccgtgatgcacgaggccctgcacaatcactacacccagaagtccctgtctctgtcccctggcaaa

SEQ ID NO: 136 - DNA, 1338 bp, Artificial Sequence
  antibody heavy chain
caggtccagctgcaagagtctggccctggactggtcaagccttccgagacactgtccatcacctgtaccgtgtccggcttctccctgtccaactacgacatctcctggatcagacagcctcctggcaaaggcctggaatggctgggagtgatttggaccggcggagccaccaactacaaccccgctctgaagtcccggctgaccatctccagagacaactccaagaaccaggtgtccctgaagatgtcctccgtgaccgctgctgataccgccgtgtactactgcgtgcgggactccaactacagatacgacgagcccttcacctactggggccagggaacactggtcaccgtgtcctctgctagcaccaaagggccgtccgtcttccccctggccccctgcagccggtcgacgtccgagtccaccgccgccctcgggtgcctggtcaaggactacttcccggagccggtaaccgtgagctggaactccggcgcgctgacctccggcgtgcacacgttccccgccgtcctgcagtcctccggcctctactccctctcgtccgtcgtcaccgtcccgagcagttccctgggcaccaagacctacacgtgcaacgtcgaccacaagccctccaacaccaaggtagacaagcgcgtcgagtccaaatacggccccccgtgcccgccctgtccggcccccgaggccgcgggcggcccctcagtgttcctgttcccgccgaagcccaaggacaccctgatgatctcgcgcacgcccgaggtcacgtgcgtggtcgtcgacgtctcacaggaagaccccgaggtgcagttcaactggtatgtcgacggcgtggaggttcacaacgcgaagaccaagccccgggaggagcagttcaacagcacataccgggtggtgtcggtcctcaccgtgctgcatcaggactggctgaacggtaaggagtacaagtgcaaggtgtccaacaagggcctcccgagcagcatagagaagaccatctccaaggcgaagggtcagccccgcgaaccgcaggtgtacaccctgccgccgagccaggaggagatgacgaagaaccaggtctccctgacgtgcctggtgaagggtttctacccctcggacatcgcggtcgaatgggaatcgaacgggcagccggagaacaactacaagaccacgccgccggtcctggactccgacgggtccttcttcctgtactcccggctgaccgtagacaagtcgcgctggcaggagggtaacgtgttcagctgcagcgtgatgcacgaggccctccacaaccactacacgcaaaagtcgctctccctgtccctgggc

SEQ ID NO: 137 - DNA, 642 bp, Artificial Sequence
  antibody light chain
gaaattgtgctgacccagtctcctgacacactgagcgtgacccctaaagaaaaagtgaccctgacctgccgggccagccagtctatcggcaccaacatccactggttccagcagaagcctggccagtctccaaagctgctgattaagtacgcctccgagtccatctccggcgtgccctctagattttccggctctggctctggcaccgacttcaccctgaccatcaactccgtggaagccgaggatgccgctacctactactgccagcagtccaactcctggccttacacctttggccagggcaccaagctggaaatcaagcggacagtggccgctccttccgtgttcatcttcccaccttccgacgagcagctgaagtccggcacagcttctgtcgtgtgcctgctgaacaacttctaccctcgggaagccaaggtgcagtggaaggtggacaatgccctgcagtccggcaactcccaagagtctgtgaccgagcaggactccaaggacagcacctacagcctgtcctccacactgaccctgtccaaggccgactacgagaagcacaaggtgtacgcctgcgaagtgacccatcagggcctgtctagccctgtgaccaagtctttcaaccggggcgagtgt

SEQ ID NO: 138 - DNA, 1842 bp, Artificial Sequence
  fusion protein
gagtccaaatacggccccccgtgcccgccctgtccggcccccgaggccgcgggcggcccctcagtgttcctgttcccgccgaagcccaaggacaccctgatgatctcgcgcacgcccgaggtcacgtgcgtggtcgtcgacgtctcacaggaagaccccgaggtgcagttcaactggtatgtcgacggcgtggaggttcacaacgcgaagaccaagccccgggaggagcagttcaacagcacataccgggtggtgtcggtcctcaccgtgctgcatcaggactggctgaacggtaaggagtacaagtgcaaggtgtccaacaagggcctcccgagcagcatagagaagaccatctccaaggcgaagggtcagccccgcgaaccgcaggtgtacaccctgccgccgagccaggaggagatgacgaagaaccaggtctccctgacgtgcctggtgaagggtttctacccctcggacatcgcggtcgaatgggaatcgaacgggcagccggagaacaactacaagaccacgccgccggtcctggactccgacgggtccttcttcctgtactcccggctgaccgtagacaagtcgcgctggcaggagggtaacgtgttcagctgcagcgtgatgcacgaggccctccacaaccactacacgcaaaagtcgctctccctgtccctgggcggaggcggaggatctggtggtggtggatctggcggcggaggttctcaggactctacctccgatctgatccccgctcctccactgtctaaggtgccactgcagcagaacttccaggacaaccagttccacggcaagtggtacgtcgtcggccaggccggaaacatcagactgagagaggacaaggaccccatcaagatgatggctaccatctacgagctgaaagaggataagtcctacgacgtcaccatggtcaagttcgacgacaaaaagtgtatgtacgacatctggaccttcgtgcccggctctcagcctggcgagtttaccctgggcaagatcaagagcttccccggccacacctcttctctcgtgcgtgtggtgtccaccaactacaaccagcacgccatggtgttcttcaagttcgtgttccagaaccgggaagagttctacatcaccctgtacggccggaccaaagagctgacctccgaactgaaagagaacttcatccggttctccaagagcctgggcctgccagagaaccacatcgtgtttccagtgcctatcgaccagtgcatcgatggcggaggcggaggatctggtggtggtggatctggcggcggaggttctcaggactctacctccgatctgatccccgctcctccactgtctaaggtgccactgcagcagaacttccaggacaaccagttccacggcaagtggtacgtcgtcggccaggccggaaacatcagactgagagaggacaaggaccccatcaagatgatggctaccatctacgagctgaaagaggataagtcctacgacgtcaccatggtcaagttcgacgacaaaaagtgtatgtacgacatctggaccttcgtgcccggctctcagcctggcgagtttaccctgggcaagatcaagagcttccccggccacacctcttctctcgtgcgtgtggtgtccaccaactacaaccagcacgccatggtgttcttcaagttcgtgttccagaaccgggaagagttctacatcaccctgtacggccggaccaaagagctgacctccgaactgaaagagaacttcatccggttctccaagagcctgggcctgccagagaaccacatcgtgttccctgtgcctatcgatcagtgtatcgacggc

SEQ ID NO: 139 - DNA, 1266 bp, Artificial Sequence
  fusion protein
gagagcaagtacggccctccctgccccccctgccctgcccctgaagccgcgggcggaccttccgtgtttctgttccccccgaagcccaaggacaccctgatgatctcccggacccccgaagtgacctgcgtggtggtggacgtgtcccaggaagatccagaggtgcagttcaactggtatgttgacggcgtggaagtgcacaacgccaagaccaagcccagagaggaacagttcaactccacctaccgggtggtgtccgtgctgaccgtgctgcaccaggactggctgaacggcaaagagtacaagtgcaaggtgtccaacaagggcctgccctccagcatcgaaaagaccatctccaaggccaagggccagccccgcgagccccaggtgtacaccctgccccctagccaggaagagatgaccaagaaccaggtgtccctgacctgtctggtgaaaggcttctacccctccgacattgccgtggaatgggagtccaacggccagcccgagaacaactacaagaccaccccccctgtgctggactccgacggctccttcttcctgtactctcggctgacagtggataagtcccggtggcaggaaggcaatgtgttctcctgcagcgtgatgcacgaggccctgcacaaccactatacccagaagtccctgtccctgagcctgggcaagggcggcggcggatccggcggcggcggctctggcggcggcggctctcaggactctacatccgatctgatccccgctcctccactgtccaaggtgcctctgcaacagaactttcaggacaaccagtttcatggcaagtggtatgtggtgggccaggctggcaatatcagactgagggaggataaggaccctatcaagatgatggccacaatctacgagctgaaggaggacaagtcttacgatgtgacaatggtgaagttcgacgacaagaagtgcatgtacgacatctggacattcgtgccaggctcccagcctggcgagtttacactgggcaagatcaagtccttcccaggccatacctccagcctggtgcgggtggtgtccacaaactataaccagcatgctatggtgtttttcaagttcgtgttccagaatcgggaggagttctacatcaccctgtacggccggaccaaggagctgacatctgagctgaaggagaacttcatcagattttccaagagcctgggcctgcctgagaaccacatcgtgtttcccgtgccaatcgatcagtgtatcgacggc

SEQ ID NO: 140 - DNA, 1917 bp, Artificial Sequence
  fusion protein
caggtccagctgcaagagtctggccctggactggtcaagccttccgagacactgtccatcacctgtaccgtgtccggcttctccctgtccaactacgacatctcctggatcagacagcctcctggcaaaggcctggaatggctgggagtgatttggaccggcggagccaccaactacaaccccgctctgaagtcccggctgaccatctccagagacaactccaagaaccaggtgtccctgaagatgtcctccgtgaccgctgctgataccgccgtgtactactgcgtgcgggactccaactacagatacgacgagcccttcacctactggggccagggaacactggtcaccgtgtcctctgctagcaccaaagggccgtccgtcttccccctggccccctgcagccggtcgacgtccgagtccaccgccgccctcgggtgcctggtcaaggactacttcccggagccggtaaccgtgagctggaactccggcgcgctgacctccggcgtgcacacgttccccgccgtcctgcagtcctccggcctctactccctctcgtccgtcgtcaccgtcccgagcagttccctgggcaccaagacctacacgtgcaacgtcgaccacaagccctccaacaccaaggtagacaagcgcgtcgagtccaaatacggccccccgtgcccgccctgtccggcccccgaggccgcgggcggcccctcagtgttcctgttcccgccgaagcccaaggacaccctgatgatctcgcgcacgcccgaggtcacgtgcgtggtcgtcgacgtctcacaggaagaccccgaggtgcagttcaactggtatgtcgacggcgtggaggttcacaacgcgaagaccaagccccgggaggagcagttcaacagcacataccgggtggtgtcggtcctcaccgtgctgcatcaggactggctgaacggtaaggagtacaagtgcaaggtgtccaacaagggcctcccgagcagcatagagaagaccatctccaaggcgaagggtcagccccgcgaaccgcaggtgtacaccctgccgccgagccaggaggagatgacgaagaaccaggtctccctgacgtgcctggtgaagggtttctacccctcggacatcgcggtcgaatgggaatcgaacgggcagccggagaacaactacaagaccacgccgccggtcctggactccgacgggtccttcttcctgtactcccggctgaccgtagacaagtcgcgctggcaggagggtaacgtgttcagctgcagcgtgatgcacgaggccctccacaaccactacacgcaaaagtcgctctccctgtccctgggcggaggcggaggatctggtggtggtggatctggcggcggaggttctcaggactctacctccgatctgatccccgctcctccactgtctaaggtgccactgcagcagaacttccaggacaaccagttccacggcaagtggtacgtcgtcggccaggccggaaacatcagactgagagaggacaaggaccccatcaagatgatggctaccatctacgagctgaaagaggataagtcctacgacgtcaccatggtcaagttcgacgacaaaaagtgtatgtacgacatctggaccttcgtgcccggctctcagcctggcgagtttaccctgggcaagatcaagagcttccccggccacacctcttctctcgtgcgtgtggtgtccaccaactacaaccagcacgccatggtgttcttcaagttcgtgttccagaaccgggaagagttctacatcaccctgtacggccggaccaaagagctgacctccgaactgaaagagaacttcatccggttctccaagagcctgggcctgccagagaaccacatcgtgttccctgtgcctatcgaccagtgcatcgatggc

SEQ ID NO: 141 - DNA, 1221 bp, Artificial Sequence
  fusion protein
gaaattgtgctgacccagtctcctgacacactgagcgtgacccctaaagaaaaagtgaccctgacctgccgggccagccagtctatcggcaccaacatccactggttccagcagaagcctggccagtctccaaagctgctgattaagtacgcctccgagtccatctccggcgtgccctctagattttccggctctggctctggcaccgacttcaccctgaccatcaactccgtggaagccgaggatgccgctacctactactgccagcagtccaactcctggccttacacctttggccagggcaccaagctggaaatcaagcggacagtggccgctccttccgtgttcatcttcccaccttccgacgagcagctgaagtccggcacagcttctgtcgtgtgcctgctgaacaacttctaccctcgggaagccaaggtgcagtggaaggtggacaatgccctgcagtccggcaactcccaagagtctgtgaccgagcaggactccaaggacagcacctacagcctgtcctccacactgaccctgtccaaggccgactacgagaagcacaaggtgtacgcctgcgaagtgacccatcagggcctgtctagccctgtgaccaagtctttcaaccggggcgagtgtggtggcggaggatctggcggaggtggaagcggcggaggcggatctcaagactctacctccgatctgatccccgctcctccactgtctaaggtgccactgcagcagaacttccaggacaaccagttccacggcaagtggtacgtcgtcggccaggccggaaacatcagactgagagaggacaaggaccccatcaagatgatggctaccatctacgagctgaaagaggataagtcctacgacgtcaccatggtcaagttcgacgacaaaaagtgtatgtacgacatctggaccttcgtgcccggctctcagcctggcgagtttaccctgggcaagatcaagagcttccccggccacacctcttctctcgtgcgtgtggtgtccaccaactacaaccagcacgccatggtgttcttcaagttcgtgttccagaaccgggaagagttctacatcaccctgtacggccggaccaaagagctgacctccgaactgaaagagaacttcatccggttctccaagagcctgggcctgcctgagaaccacatcgtgttccctgtgcctatcgaccagtgcatcgatggc

SEQ ID NO: 142 - DNA, 1917 bp, Artificial Sequence
  fusion protein
caggactccacctccgatctgatccctgctcctccactgtctaaggtgcccctgcagcagaacttccaggacaaccagttccacggcaagtggtacgtcgtcggccaggccggaaacatcagactgagagaggacaaggaccccatcaagatgatggctaccatctacgagctgaaagaggataagtcctacgacgtcaccatggtcaagttcgacgacaaaaagtgtatgtacgacatctggaccttcgtgcccggctctcagcctggcgagtttaccctgggcaagatcaagagcttccccggccacacctcttctctcgtgcgtgtggtgtccaccaactacaaccagcacgccatggtgttcttcaagttcgtgttccagaaccgggaagagttctacatcaccctgtacggccggaccaaagagctgacctccgaactgaaagagaacttcatccggttctccaagagcctgggcctgcctgagaaccacatcgtgttccctgtgcctatcgaccagtgcatcgatggcggaggcggaggatctggtggtggtggatctggcggcggaggttctcaggtccagctgcaagagtctggccctggactggtcaagccttccgagacactgtccatcacctgtaccgtgtccggcttctccctgtccaactacgacatctcctggatcagacagcctcctggcaaaggcctggaatggctgggagtgatttggaccggcggagccaccaactacaaccccgctctgaagtcccggctgaccatctccagagacaactccaagaaccaggtgtccctgaagatgtcctccgtgaccgctgctgataccgccgtgtactactgcgtgcgggactccaactacagatacgacgagcccttcacctactggggccagggaacactggtcaccgtgtcctctgctagcaccaaagggccgtccgtcttccccctggccccctgcagccggtcgacgtccgagtccaccgccgccctcgggtgcctggtcaaggactacttcccggagccggtaaccgtgagctggaactccggcgcgctgacctccggcgtgcacacgttccccgccgtcctgcagtcctccggcctctactccctctcgtccgtcgtcaccgtcccgagcagttccctgggcaccaagacctacacgtgcaacgtcgaccacaagccctccaacaccaaggtagacaagcgcgtcgagtccaaatacggccccccgtgcccgccctgtccggcccccgaggccgcgggcggcccctcagtgttcctgttcccgccgaagcccaaggacaccctgatgatctcgcgcacgcccgaggtcacgtgcgtggtcgtcgacgtctcacaggaagaccccgaggtgcagttcaactggtatgtcgacggcgtggaggttcacaacgcgaagaccaagccccgggaggagcagttcaacagcacataccgggtggtgtcggtcctcaccgtgctgcatcaggactggctgaacggtaaggagtacaagtgcaaggtgtccaacaagggcctcccgagcagcatagagaagaccatctccaaggcgaagggtcagccccgcgaaccgcaggtgtacaccctgccgccgagccaggaggagatgacgaagaaccaggtctccctgacgtgcctggtgaagggtttctacccctcggacatcgcggtcgaatgggaatcgaacgggcagccggagaacaactacaagaccacgccgccggtcctggactccgacgggtccttcttcctgtactcccggctgaccgtagacaagtcgcgctggcaggagggtaacgtgttcagctgcagcgtgatgcacgaggccctccacaaccactacacgcaaaagtcgctctccctgtccctgggc

SEQ ID NO: 143 - DNA, 1221 bp, Artificial Sequence
  fusion protein
caggattctacctccgatctgatccccgctcctccactgtctaaggtgcccctgcagcagaacttccaggacaaccagttccacggcaagtggtacgtcgtcggccaggccggaaacatcagactgagagaggacaaggaccccatcaagatgatggctaccatctacgagctgaaagaggataagtcctacgacgtcaccatggtcaagttcgacgacaaaaagtgtatgtacgacatctggaccttcgtgcccggctctcagcctggcgagtttaccctgggcaagatcaagagcttccccggccacacctcttctctcgtgcgtgtggtgtccaccaactacaaccagcacgccatggtgttcttcaagttcgtgttccagaaccgggaagagttctacatcaccctgtacggccggaccaaagagctgacctccgaactgaaagagaacttcatccggttctccaagagcctgggcctgcctgagaaccacatcgtgttccctgtgcctatcgaccagtgcatcgatggcggaggcggaggatctggcggaggtggaagcggaggcggtggatctgaaattgtgctgacccagtctcctgacacactgagcgtgacccctaaagaaaaagtgaccctgacctgccgggccagccagtctatcggcaccaacatccactggttccagcagaagcctggccagtctccaaagctgctgattaagtacgcctccgagtccatctccggcgtgccctctagattttccggctctggctctggcaccgacttcaccctgaccatcaactccgtggaagccgaggatgccgctacctactactgccagcagtccaactcctggccttacacctttggccagggcaccaagctggaaatcaagcggacagtggccgctccttccgtgttcatcttcccaccttccgacgagcagctgaagtccggcacagcttctgtcgtgtgcctgctgaacaacttctaccctcgggaagccaaggtgcagtggaaggtggacaatgccctgcagtccggcaactcccaagagtctgtgaccgagcaggactccaaggacagcacctacagcctgtcctccacactgaccctgtccaaggccgactacgagaagcacaaggtgtacgcctgcgaagtgacccatcagggcctgtctagccctgtgaccaagtctttcaaccggggcgagtgt

SEQ ID NO: 144 - DNA, 2496 bp, Artificial Sequence
  fusion protein
caggtccagctgcaagagtctggccctggactggtcaagccttccgagacactgtccatcacctgtaccgtgtccggcttctccctgtccaactacgacatctcctggatcagacagcctcctggcaaaggcctggaatggctgggagtgatttggaccggcggagccaccaactacaaccccgctctgaagtcccggctgaccatctccagagacaactccaagaaccaggtgtccctgaagatgtcctccgtgaccgctgctgataccgccgtgtactactgcgtgcgggactccaactacagatacgacgagcccttcacctactggggccagggaacactggtcaccgtgtcctctgctagcaccaaagggccgtccgtcttccccctggccccctgcagccggtcgacgtccgagtccaccgccgccctcgggtgcctggtcaaggactacttcccggagccggtaaccgtgagctggaactccggcgcgctgacctccggcgtgcacacgttccccgccgtcctgcagtcctccggcctctactccctctcgtccgtcgtcaccgtcccgagcagttccctgggcaccaagacctacacgtgcaacgtcgaccacaagccctccaacaccaaggtagacaagcgcgtcgagtccaaatacggccccccgtgcccgccctgtccggcccccgaggccgcgggcggcccctcagtgttcctgttcccgccgaagcccaaggacaccctgatgatctcgcgcacgcccgaggtcacgtgcgtggtcgtcgacgtctcacaggaagaccccgaggtgcagttcaactggtatgtcgacggcgtggaggttcacaacgcgaagaccaagccccgggaggagcagttcaacagcacataccgggtggtgtcggtcctcaccgtgctgcatcaggactggctgaacggtaaggagtacaagtgcaaggtgtccaacaagggcctcccgagcagcatagagaagaccatctccaaggcgaagggtcagccccgcgaaccgcaggtgtacaccctgccgccgagccaggaggagatgacgaagaaccaggtctccctgacgtgcctggtgaagggtttctacccctcggacatcgcggtcgaatgggaatcgaacgggcagccggagaacaactacaagaccacgccgccggtcctggactccgacgggtccttcttcctgtactcccggctgaccgtagacaagtcgcgctggcaggagggtaacgtgttcagctgcagcgtgatgcacgaggccctccacaaccactacacgcaaaagtcgctctccctgtccctgggcggaggcggaggatctggtggtggtggatctggcggcggaggttctcaggactctacctccgatctgatccccgctcctccactgtctaaggtgccactgcagcagaacttccaggacaaccagttccacggcaagtggtacgtcgtcggccaggccggaaacatcagactgagagaggacaaggaccccatcaagatgatggctaccatctacgagctgaaagaggataagtcctacgacgtcaccatggtcaagttcgacgacaaaaagtgtatgtacgacatctggaccttcgtgcccggctctcagcctggcgagtttaccctgggcaagatcaagagcttccccggccacacctcttctctcgtgcgtgtggtgtccaccaactacaaccagcacgccatggtgttcttcaagttcgtgttccagaaccgggaagagttctacatcaccctgtacggccggaccaaagagctgacctccgaactgaaagagaacttcatccggttctccaagagcctgggcctgccagagaaccacatcgtgtttccagtgcctatcgaccagtgcatcgatggcggaggcggaggatctggtggtggtggatctggcggcggaggttctcaggactctacctccgatctgatccccgctcctccactgtctaaggtgccactgcagcagaacttccaggacaaccagttccacggcaagtggtacgtcgtcggccaggccggaaacatcagactgagagaggacaaggaccccatcaagatgatggctaccatctacgagctgaaagaggataagtcctacgacgtcaccatggtcaagttcgacgacaaaaagtgtatgtacgacatctggaccttcgtgcccggctctcagcctggcgagtttaccctgggcaagatcaagagcttccccggccacacctcttctctcgtgcgtgtggtgtccaccaactacaaccagcacgccatggtgttcttcaagttcgtgttccagaaccgggaagagttctacatcaccctgtacggccggaccaaagagctgacctccgaactgaaagagaacttcatccggttctccaagagcctgggcctgccagagaaccacatcgtgttccctgtgcctatcgatcagtgtatcgacggc

SEQ ID NO: 145 - protein, 442 aa, Artificial Sequence
  antibody heavy chain
EVQLVQSGAEVKKPGESLRISCKGSGYSFSTYWISWVRQMPGKGLEWMGKIYPGDSYTNYSPSFQGQVTISADKSISTAYLQWSSLKASDTAMYYCARGYGIFDYWGQGTLVTVSSASTKGPSVFPLAPCSRSTSESTAALGCLVKDYFPEPVTVSWNSGALTSGVHTFPAVLQSSGLYSLSSVVTVPSSNFGTQTYTCNVDHKPSNTKVDKTVERKCCVECPPCPAPPVAGPSVFLFPPKPKDTLMISRTPEVTCVVVDVSHEDPEVQFNWYVDGVEVHNAKTKPREEQFNSTFRVVSVLTVVHQDWLNGKEYKCKVSNKGLPAPIEKTISKTKGQPREPQVYTLPPSREEMTKNQVSLTCLVKGFYPSDIAVEWESNGQPENNYKTTPPMLDSDGSFFLYSKLTVDKSRWQQGNVFSCSVMHEALHNHYTQKSLSLSPGK

SEQ ID NO: 146 - protein, 214 aa, Artificial Sequence
  antibody light chain
SYELTQPPSVSVSPGQTASITCSGDNIGDQYAHWYQQKPGQSPVLVIYQDKNRPSGIPERFSGSNSGNTATLTISGTQAMDEADYYCATYTGFGSLAVFGGGTKLTVLGQPKAAPSVTLFPPSSEELQANKATLVCLISDFYPGAVTVAWKADSSPVKAGVETTTPSKQSNNKYAASSYLSLTPEQWKSHRSYSCQVTHEGSTVEKTVAPTECS

SEQ ID NO: 147 - protein, 472 aa, Artificial Sequence
  fusion protein
EVQLLESGGGEVQPGGSLRLSCAASGGIFAIKPISWYRQAPGKQREWVSTTTSSGATNYAESVKGRFTISRDNAKNTLYLQMSSLRAEDTAVYYCNVFEYWGQGTLVTVKPGGGGDKTHTCPPCPAPGGPSVFLFPPKPKDTLMISRTPEVTCVVVDVSHEDPEVKFNWYVDGVEVHNAKTKPREEQYNSTYRVVSVLTVLHQDWLNGKEYKCKVSNKALPAPIEKTISKAKGQPREPQVYTLPPSRDELTKNQVSLTCLVKGFYPSDIAVEWESNGQPENNYKTTPPVLDSDGSFFLYSKLTVDKSRWQQGNVFSCSVMHEALHNHYTQKSLSLSPGSGGGGSGGGGSEVQLLESGGGEVQPGGSLRLSCAASGFSFSINAMGWYRQAPGKRREFVAAIESGRNTVYAESVKGRFTISRDNAKNTVYLQMSSLRAEDTAVYYCGLLKGNRVVSPSVAYWGQGTLVTVKPGG

SEQ ID NO: 148 - protein, 466 aa, Artificial Sequence
  fusion protein
EVQLLESGGGEVQPGGSLRLSCAASGGIFAIKPISWYRQAPGKQREWVSTTTSSGATNYAESVKGRFTISRDNAKNTLYLQMSSLRAEDTAVYYCNVFEYWGQGTLVTVKPGGSGGSEVQLLESGGGEVQPGGSLRLSCAASGFSFSINAMGWYRQAPGKRREFVAAIESGRNTVYAESVKGRFTISRDNAKNTVYLQMSSLRAEDTAVYYCGLLKGNRVVSPSVAYWGQGTLVTVKPGGGGDKTHTCPPCPAPGGPSVFLFPPKPKDTLMISRTPEVTCVVVDVSHEDPEVKFNWYVDGVEVHNAKTKPREEQYNSTYRVVSVLTVLHQDWLNGKEYKCKVSNKALPAPIEKTISKAKGQPREPQVYTLPPSRDELTKNQVSLTCLVKGFYPSDIAVEWESNGQPENNYKTTPPVLDSDGSFFLYSKLTVDKSRWQQGNVFSCSVMHEALHNHYTQKSLSLSPGK